European Patent Specification EP 3 186 371 B1, published August 14, 2024. Title: Administration of kynurenine depleting enzymes for tumor therapy. Applicant: Board of Regents, The University of Texas System. Application Unknown. The sequence listing filed with the application follows.

SEQUENCE LISTING (93 sequences)

SEQ ID NO: 1 - DNA, 1347 bp, Artificial Sequence
  Synthetic polynucleotide
tctagaaataattttgtttaactttaaggaaaacattaaaataaggaggtagcaaatgggcggtcatcatcaccaccatcatgggagcggcaccacccgcaacgattgcctggcgctggatgcgcaggatagcctggcaccgctgcgtcagcagtttgcgctgccggaaggtgttatttatctggatggcaacagcctgggtgcgcgtccggttgcggcgctggcgcgtgcgcaggcggtgattgcggaagaatggggcaacggcctgattcgcagctggaacagcgcgggctggcgcgatctgagcgaacgcctgggcaaccgcctggcgaccctgattggcgcgcgcgatggcgaagtggtggtgaccgataccaccagcattaacctgtttaaagtgctgagcgcggcgctgcgcgtgcaggcgacccgcagcccggaacgccgcgtgattgtgaccgaaaccagcaactttccgaccgatctgtatattgcggaaggcctggcggatatgctgcagcagggctataccctgcgcctggtggatagcccggaagaactgccgcaggcgattgatcaggataccgcggtggtgatgctgacccatgtgaactataaaaccggctatatgcatgatatgcaggcgctgaccgcgctgagccatgaatgcggcgcgctggcgatttgggatctggcgcatagcgcgggcgcggtgccggtggatctgcatcaggcgggcgcggattatgcgattggctgcacctataaatatctgaacggcggcccgggcagccaggcgtttgtgtgggtgagcccgcagctgtgcgatctggtgccgcagccgctgtctggttggtttggccatagccgccagtttgcgatggaaccgcgctatgaaccgagcaacggcattgcgcgctatctgtgcggcacccagccgattaccagcctggcgatggtggaatgcggcctggatgtgtttgcgcagaccgatatggcgagcctgcgccgcaaaagcctggcgctgaccgatctgtttattgaactggtggaacagcgctgcgcggcgcatgaactgaccctggtgaccccgcgcgaacatgcgaaacgcggcagccatgtgagctttgaacatccggaaggctatgcggtgattcaggcgctgattgatcgcggcgtgattggcgattatcgcgaaccgcgcattatgcgctttggctttaccccgctgtataccacctttaccgaagtgtgggatgcggtgcagattctgggcgaaattctggatcgcaaaacctgggcgcaggcgcagtttcaggtgcgccatagcgtgacctagtaggatcc

SEQ ID NO: 2 - DNA, 1497 bp, Artificial Sequence
  Synthetic polynucleotide
tctagaaataattttgtttaactttaaggacaaatcaggacacagttaaggaggtaaaatatgggcggtcatcatcaccaccatcatgggagcggcgaaccgagctcccttgaacttccggccgataccgtgcaacggatagcggcggaattgaaatgtcacccgaccgacgaacgcgtcgcgttacatctggatgaggaagacaagctgcgtcacttccgcgagtgcttttacattccgaaaattcaggatctgccgccagtggacttgagcctggtcaacaaagacgagaacgccatctacttcctgggcaatagcctgggcctgcaaccaaagatggtgaaaacctatcttgaggaggagcttgacaaatgggcgaagatcgcggcctacggccatgaagtcggcaagcgtccctggattaccggcgatgagtcaatcgttggcttgatgaaggatatcgtcggcgcgaacgagaaagaaattgcgctgatgaacgcgctgaccgtgaatctgcatctgctgatgctgtcattctttaagcccaccccgaagcgctacaaaatcctgctggaagcgaaagcgtttcccagcgatcattatgcgatagaaagccagctgcaactgcacggcctgaatatcgaggagagcatgcgtatgataaaaccgcgcgaaggtgaggagaccctgcggattgaggacatcctggaggtgatcgagaaggagggcgacagtatcgcggtgatacttttcagcggcgtgcatttctacacgggccaacacttcaatatcccggccattaccaaagccggccaggcgaaagggtgctatgtaggctttgatctggcgcatgcagtgggcaacgtcgaactgtatcttcatgattggggcgttgattttgcgtgctggtgcagctataagtatctgaatgccggggccggtgggattgcgggagcctttattcatgagaaacacgcgcataccattaaaccggcgctggttggctggtttgggcacgaactgagcacccgcttcaagatggataacaaactgcaattgattccgggcgtgtgcggctttcgtattagcaaccccccgattctgctggtctgcagcctgcacgcgtctctggagattttcaagcaggcgaccatgaaagcgctgcgtaagaaaagtgtgcttctgacgggctacctggagtacctgataaagcacaactacggcaaggataaggcggccacgaagaagccggttgtgaacattatcaccccgtctcatgtggaagaacgtggctgccaactgacgataacgttcagcgtgccaaacaaggacgtgttccaagagctggagaagcgtggcgtggtgtgtgataaacgtaatccgaatggcattcgtgtggcgcctgtgccgctgtacaacagcttccacgacgtgtataagttcaccaacctgctgacgagcattctggacagtgcggaaaccaaaaactagggatcc

SEQ ID NO: 3 - DNA, 1492 bp, Artificial Sequence
  Synthetic polynucleotide
tctagaaataattttgtttaactttaagaacacggtcgggaatataaggaggtaaaatatgggcggtcatcatcaccaccatcatgggagcggcgagccgagcccgctggaactgccggttgacgcggtacgtcgtattgcggcagaactgaactgtgacccgaccgatgaacgtgtggcgctgcgtctcgacgaagaggacaagctctctcacttccgtaactgcttctatatccctaaaatgcgtgacctgccgagcatcgatctgtctctggtttctgaagacgacgacgcgatttacttcctgggtaactctctgggtctgcagccaaaaatggttcgtacctacctggaggaagagctggacaaatgggcgaaaatgggtgcctacggccatgatgtgggcaaacgcccgtggatcgtcggcgacgaaagcattgtgtctctcatgaaggacattgttggtgcacacgagaaagaaattgcgctgatgaatgctctgaccatcaacctgcacctgctgctcctgtctttcttcaagccgaccccgaagcgtcataaaatcctgctcgaggctaaagcgttcccgtctgatcactacgcgatcgaatctcaaatccaactgcacggtctggacgttgagaagtctatgcgtatggttaagccgcgtgaaggcgaggagaccctccgtatggaagacatcctcgaagttatcgaagaagaaggtgactctatcgcagttattctgttctctggcctgcacttttacaccggtcaactgttcaatatcccggcaatcaccaaagcgggccacgcgaaaggttgcttcgttggtttcgacctggcccatgcggttggtaacgtggagctgcgcctccacgactggggtgttgactttgcgtgctggtgctcttacaaatacctgaactctggtgcgggtggtctcgcgggtgcgttcgtccacgaaaaacacgcgcacaccgttaaaccggcgctggttggctggttcggccacgacctctctacgcgtttcaacatggacaacaaactccagctgatcccaggcgccaacggtttccgtatctctaacccgccgatcctcctggtttgctctctgcacgcgtctctcgaggttttccagcaggcgaccatgaccgccctgcgccgtaaatctattctcctgacgggttatctggaatacatgctgaagcactaccactctaaagacaacacggaaaacaaaggtccgatcgttaacatcatcaccccgtctcgtgcggaagaacgtggctgccaactgaccctgaccttctctattccgaaaaaatctgttttcaaagaactggagaaacgtggtgttgtttgcgacaaacgtgaaccggacggtatccgcgttgctccggtcccgctgtacaactctttccatgacgtttataagttcattcgtctgctcacctccatcctggactctagcgaacgctcctaaggatcc

SEQ ID NO: 4 - DNA, 1251 bp, Pseudomonas fluorescens
atgaccacccgcaacgattgcctggcgctggatgcgcaggatagcctggcaccgctgcgtcagcagtttgcgctgccggaaggtgttatttatctggatggcaacagcctgggtgcgcgtccggttgcggcgctggcgcgtgcgcaggcggtgattgcggaagaatggggcaacggcctgattcgcagctggaacagcgcgggctggcgcgatctgagcgaacgcctgggcaaccgcctggcgaccctgattggcgcgcgcgatggcgaagtggtggtgaccgataccaccagcattaacctgtttaaagtgctgagcgcggcgctgcgcgtgcaggcgacccgcagcccggaacgccgcgtgattgtgaccgaaaccagcaactttccgaccgatctgtatattgcggaaggcctggcggatatgctgcagcagggctataccctgcgcctggtggatagcccggaagaactgccgcaggcgattgatcaggataccgcggtggtgatgctgacccatgtgaactataaaaccggctatatgcatgatatgcaggcgctgaccgcgctgagccatgaatgcggcgcgctggcgatttgggatctggcgcatagcgcgggcgcggtgccggtggatctgcatcaggcgggcgcggattatgcgattggctgcacctataaatatctgaacggcggcccgggcagccaggcgtttgtgtgggtgagcccgcagctgtgcgatctggtgccgcagccgctgtctggttggtttggccatagccgccagtttgcgatggaaccgcgctatgaaccgagcaacggcattgcgcgctatctgtgcggcacccagccgattaccagcctggcgatggtggaatgcggcctggatgtgtttgcgcagaccgatatggcgagcctgcgccgcaaaagcctggcgctgaccgatctgtttattgaactggtggaacagcgctgcgcggcgcatgaactgaccctggtgaccccgcgcgaacatgcgaaacgcggcagccatgtgagctttgaacatccggaaggctatgcggtgattcaggcgctgattgatcgcggcgtgattggcgattatcgcgaaccgcgcattatgcgctttggctttaccccgctgtataccacctttaccgaagtgtgggatgcggtgcagattctgggcgaaattctggatcgcaaaacctgggcgcaggcgcagtttcaggtgcgccatagcgtgacctag

SEQ ID NO: 5 - DNA, 1398 bp, Homo sapiens
atggaaccgagctcccttgaacttccggccgataccgtgcaacggatagcggcggaattgaaatgtcacccgaccgacgaacgcgtcgcgttacatctggatgaggaagacaagctgcgtcacttccgcgagtgcttttacattccgaaaattcaggatctgccgccagtggacttgagcctggtcaacaaagacgagaacgccatctacttcctgggcaatagcctgggcctgcaaccaaagatggtgaaaacctatcttgaggaggagcttgacaaatgggcgaagatcgcggcctacggccatgaagtcggcaagcgtccctggattaccggcgatgagtcaatcgttggcttgatgaaggatatcgtcggcgcgaacgagaaagaaattgcgctgatgaacgcgctgaccgtgaatctgcatctgctgatgctgtcattctttaagcccaccccgaagcgctacaaaatcctgctggaagcgaaagcgtttcccagcgatcattatgcgatagaaagccagctgcaactgcacggcctgaatatcgaggagagcatgcgtatgataaaaccgcgcgaaggtgaggagaccctgcggattgaggacatcctggaggtgatcgagaaggagggcgacagtatcgcggtgatacttttcagcggcgtgcatttctacacgggccaacacttcaatatcccggccattaccaaagccggccaggcgaaagggtgctatgtaggctttgatctggcgcatgcagtgggcaacgtcgaactgtatcttcatgattggggcgttgattttgcgtgctggtgcagctataagtatctgaatgccggggccggtgggattgcgggagcctttattcatgagaaacacgcgcataccattaaaccggcgctggttggctggtttgggcacgaactgagcacccgcttcaagatggataacaaactgcaattgattccgggcgtgtgcggctttcgtattagcaaccccccgattctgctggtctgcagcctgcacgcgtctctggagattttcaagcaggcgaccatgaaagcgctgcgtaagaaaagtgtgcttctgacgggctacctggagtacctgataaagcacaactacggcaaggataaggcggccacgaagaagccggttgtgaacattatcaccccgtctcatgtggaagaacgtggctgccaactgacgataacgttcagcgtgccaaacaaggacgtgttccaagagctggagaagcgtggcgtggtgtgtgataaacgtaatccgaatggcattcgtgtggcgcctgtgccgctgtacaacagcttccacgacgtgtataagttcaccaacctgctgacgagcattctggacagtgcggaaaccaaaaactag

SEQ ID NO: 6 - DNA, 1395 bp, Mus musculus
atggagccgagcccgctggaactgccggttgacgcggtacgtcgtattgcggcagaactgaactgtgacccgaccgatgaacgtgtggcgctgcgtctcgacgaagaggacaagctctctcacttccgtaactgcttctatatccctaaaatgcgtgacctgccgagcatcgatctgtctctggtttctgaagacgacgacgcgatttacttcctgggtaactctctgggtctgcagccaaaaatggttcgtacctacctggaggaagagctggacaaatgggcgaaaatgggtgcctacggccatgatgtgggcaaacgcccgtggatcgtcggcgacgaaagcattgtgtctctcatgaaggacattgttggtgcacacgagaaagaaattgcgctgatgaatgctctgaccatcaacctgcacctgctgctcctgtctttcttcaagccgaccccgaagcgtcataaaatcctgctcgaggctaaagcgttcccgtctgatcactacgcgatcgaatctcaaatccaactgcacggtctggacgttgagaagtctatgcgtatggttaagccgcgtgaaggcgaggagaccctccgtatggaagacatcctcgaagttatcgaagaagaaggtgactctatcgcagttattctgttctctggcctgcacttttacaccggtcaactgttcaatatcccggcaatcaccaaagcgggccacgcgaaaggttgcttcgttggtttcgacctggcccatgcggttggtaacgtggagctgcgcctccacgactggggtgttgactttgcgtgctggtgctcttacaaatacctgaactctggtgcgggtggtctcgcgggtgcgttcgtccacgaaaaacacgcgcacaccgttaaaccggcgctggttggctggttcggccacgacctctctacgcgtttcaacatggacaacaaactccagctgatcccaggcgccaacggtttccgtatctctaacccgccgatcctcctggtttgctctctgcacgcgtctctcgaggttttccagcaggcgaccatgaccgccctgcgccgtaaatctattctcctgacgggttatctggaatacatgctgaagcactaccactctaaagacaacacggaaaacaaaggtccgatcgttaacatcatcaccccgtctcgtgcggaagaacgtggctgccaactgaccctgaccttctctattccgaaaaaatctgttttcaaagaactggagaaacgtggtgttgtttgcgacaaacgtgaaccggacggtatccgcgttgctccggtcccgctgtacaactctttccatgacgtttataagttcattcgtctgctcacctccatcctggactctagcgaacgctcctaa

SEQ ID NO: 7 - protein, 416 aa, Pseudomonas fluorescens
MTTRNDCLALDAQDSLAPLRQQFALPEGVIYLDGNSLGARPVAALARAQAVIAEEWGNGLIRSWNSAGWRDLSERLGNRLATLIGARDGEVVVTDTTSINLFKVLSAALRVQATRSPERRVIVTETSNFPTDLYIAEGLADMLQQGYTLRLVDSPEELPQAIDQDTAVVMLTHVNYKTGYMHDMQALTALSHECGALAIWDLAHSAGAVPVDLHQAGADYAIGCTYKYLNGGPGSQAFVWVSPQLCDLVPQPLSGWFGHSRQFAMEPRYEPSNGIARYLCGTQPITSLAMVECGLDVFAQTDMASLRRKSLALTDLFIELVEQRCAAHELTLVTPREHAKRGSHVSFEHPEGYAVIQALIDRGVIGDYREPRIMRFGFTPLYTTFTEVWDAVQILGEILDRKTWAQAQFQVRHSVT

SEQ ID NO: 8 - protein, 465 aa, Homo sapiens
MEPSSLELPADTVQRIAAELKCHPTDERVALHLDEEDKLRHFRECFYIPKIQDLPPVDLSLVNKDENAIYFLGNSLGLQPKMVKTYLEEELDKWAKIAAYGHEVGKRPWITGDESIVGLMKDIVGANEKEIALMNALTVNLHLLMLSFFKPTPKRYKILLEAKAFPSDHYAIESQLQLHGLNIEESMRMIKPREGEETLRIEDILEVIEKEGDSIAVILFSGVHFYTGQHFNIPAITKAGQAKGCYVGFDLAHAVGNVELYLHDWGVDFACWCSYKYLNAGAGGIAGAFIHEKHAHTIKPALVGWFGHELSTRFKMDNKLQLIPGVCGFRISNPPILLVCSLHASLEIFKQATMKALRKKSVLLTGYLEYLIKHNYGKDKAATKKPVVNIITPSHVEERGCQLTITFSVPNKDVFQELEKRGVVCDKRNPNGIRVAPVPLYNSFHDVYKFTNLLTSILDSAETKN

SEQ ID NO: 9 - protein, 464 aa, Mus musculus
MEPSPLELPVDAVRRIAAELNCDPTDERVALRLDEEDKLSHFRNCFYIPKMRDLPSIDLSLVSEDDDAIYFLGNSLGLQPKMVRTYLEEELDKWAKMGAYGHDVGKRPWIVGDESIVSLMKDIVGAHEKEIALMNALTINLHLLLLSFFKPTPKRHKILLEAKAFPSDHYAIESQIQLHGLDVEKSMRMVKPREGEETLRMEDILEVIEEEGDSIAVILFSGLHFYTGQLFNIPAITKAGHAKGCFVGFDLAHAVGNVELRLHDWGVDFACWCSYKYLNSGAGGLAGAFVHEKHAHTVKPALVGWFGHDLSTRFNMDNKLQLIPGANGFRISNPPILLVCSLHASLEVFQQATMTALRRKSILLTGYLEYMLKHYHSKDNTENKGPIVNIITPSRAEERGCQLTLTFSIPKKSVFKELEKRGVVCDKREPDGIRVAPVPLYNSFHDVYKFIRLLTSILDSSERS

SEQ ID NO: 10 - protein, 466 aa, Pongo abelii
MEPSSLELPADTVQRIAAELKCHPTDERVALHLDEEDKLRHFREYFYIPKIRDLPPVDFIISESKDENAIYFLGNSLGLQPKMVKTYLEEELDKWAKIAAYGHEVGKRPWITGDESIVGLMKDIVGANEKEIALMNALTVNLHLLMLSFFKPTPKRYKILLEAKAFPSDHYAIESQLQLHGLNIEESMRMVKPREGEETLRTEDILEVIEKEGDSIAVILFSGVHFYTGQHFNIPAITKAGQAKGCYVGFDLAHAVGNVELYLHDWGVDFACWCSYKYLNAGAGGIAGAFVHEKHAHTIKPALVGWFGHELSTRFKMDNKLQLIPGVCGFRISNPPILLVCSLHASLEIFKQATMKALRKKSILLTGYLEYLIKHSYGKDKAATKKPVVNIITPSHIEERGCQLTITFSVPNKDVFQELEKRGVVCDKRNPNGIRVAPVPLYNSFHDVYKFTNLLTSILDSAETTN

SEQ ID NO: 11 - protein, 465 aa, Macaca fascicularis
MEPSPLELPADTVQRIATELKCHPTDERVALHLDEVDKLRHFRECFYIPKIQDLPPVDLSLVNKDENAIYFLGNSLGLQPKMVKTYLEEELDKWAKIAAYGHEVGKRPWITGDESIVGLMKDIVGANEKEIALMNALTVNLHLLLLSFFKPTPKRYKILLEAKAFPSDHYAIESQLQLHGLNIEESMRMIKPREGEETLRIEDILEVIEKEGDSIAVILFSGVHFYTGQHFNIPAITKAGQAKGCYVGFDLAHAVGNVELYLHDWGVDFACWCSYKYLNAGAGGIAGAFIHEKHAHTIKPALVGWFGHELSTRFKMDNKLQLIPGVCGFRISNPPILLVCSLHASLEIFKQATMKALRKKSILLTGYLEYLIKHKYGKDKAATEKPIVNIITPSHIEERGCQLTITFSVPNKDVFQELEKRGVVCDKRNPNGIRVAPVPLYNSFHDVYKFTNLLTSILDSAETTN

SEQ ID NO: 12 - protein, 465 aa, Pan troglodytes
MEPSSVELPADTVQRIAAELKCHPTDERVALHLDEEDKLRHFRECFYIPKIQDLPPVDLSLVNKDENAIYFLGNSLGLQPKMVKTYLEEELDKWAKIAAYGHEVGKRPWITGDESIVGLMKDIVGANEKEIALMNALTVNLHLLMLSFFKPTPKRYKILLEAKAFPSDHYAIESQLQLHGLNIEESMRMIKPREGEETLRIEDILEVIEKEGDSIAVILFSGVHFYTGQHFNIPAITKAGQAKGCYVGFDLAHAVGNVELYLHDWGVDFACWCSYKYLNAGAGGIAGAFIHEKHAHTIKPALVGWFGHELSTRFKMDNKLQLIPGVCGFRISNPPILLVCSLHASLEIFKQATMKALRKKSVLLTGYLEYLIKHNYGKDKAATKKPVVNIITPSHVEERGCQLTITFSVPNKDVFQELEKRGVVCDKRNPNGIRVAPVPLYNSFHDVYKFTNLLTSILDSAETTN

SEQ ID NO: 13 - protein, 431 aa, Arenitalea lutea
MLETENIRTLSDYKLGLDYALDQDRKDELKSYRNQFHIPKDKQGDAWIYMTGNSLGLQPKQTKAYVNQELNDWANLGVEGHFEAKNPWLAYHEFLTESMAKVVGAKPIEVVVMNTLTANLHFMMVSFYKPTKTRYKILIESDAFPSDKYAVESQLRHHGFDDKEGVVLWKPRPGEELLNYDDLETILETQGDEIALIMIGGVNYYTGQYFDLKRITQLGHKQGCNVGFDCAHGAGNVALNLHDSGADFAVWCTYKYLNSGPGSLAGCFVHERHAYRKDLNRFTGWWSHNKQTRFNMRGEFDQLPGAEGWQLSNPPILSMAAIKASLDLFNEVGMDKLINKSKKLTGYFEYLLKQLGEDTIRIITPKRSEERGCQLSIQVKNADKSLHNKLTEVGIISDWREPDVIRCAPVPLYNSFEDVYRLVEKLKGILK

SEQ ID NO: 14 - protein, 429 aa, Belliella Baltica DSM 15883
MSNQINFEYSLDFAQKMDEKDPLKSFRSKFFFPKVEDKEAIYFCGNSLGLQPKTTQNYIQKELSNWAEMAVDGHFHGEDAWYHIRKKSKPALAEIVGAHEHEVVAMNNLTSNLHFLMVSFYRPNAKRFKIITEAGAFPSDMYMLETQVKFHGLDPNKAIVELAPRDGEHTLRTEDILQSIKEQGEELALVMMAGLQYYTGQVFDMKAIAQAVKDEGAFVGFDLAHAAGNVPLALHDWGVDFATWCSYKYMNSGPGNVSGIFVHENHAEKPDMIRFAGWWGHDEGERFKMEKGFKPMFGADGWQLANSNVLALAAHQASLDIFQQAGIKTLREKSETLTSYLEFLIQKISGNSGVLEIITPKNINERGCQLSLLVHKGGKAVFDEFYKNGIVGDWRNPNVIRIAPTPLYNSYEDVFRFAKILEQSLQKFA

SEQ ID NO: 15 - protein, 422 aa, Bizionia argentinensis
MSNFKTGIDFAKEQDENDTLSCYRNQFHIPKDKQGNDMIYLCGNSLGLQPKATKDYINQELEDWANLGVEGHTHAKNPWLGYHEFLTDSMAKVVGAKPIEVVVMNTLTANLHFMMVSFYKPTIERYKIIIEADAFPSDKYAVESQLRHHGYDDKEGLLLWKAREGEELLRYEDLEAILKEHGDDVALVMIGGVNYYTGQFFDLKRITELGHKHGCMVGFDCAHGAGNVELNLHDSGADFAVWCTYKYLNSGPGSLGGCFVHERHAHNKRLNRFTGWWSHNKETRFKMRDEFDAIPGAEGWQLSNPPILSMAAIKASLDIFEEIGMKKLNEKSRALTAYFEFLLKQVGDDSIRIITPENPDERGCQLSIQVKNADRSLHDKLTDAGVISDWREPDVIRCAPIPLYNSYQDVYHMVERLKNILE

SEQ ID NO: 16 - protein, 431 aa, Candidatus Entotheonella sp. TSY2
MTAFHAHFQPTREAALALDASDELAPYRDQFCLPQTQGQPVVYLCGHSLGLQPKTVREYIDEELQDWAALGVEGHFHARRPWLSYHEILTAQTARLAGAKPAEVVVMNSLTVNMHLMLVSFYRPTPERFKILIEADAFPSDRYAAESHLRWHGYDPQDALLTLQPRPGEAAVRQEDIAAFLHREGETIALVWLGGVNYYTGQVFDMAEITAIGHAQGCVVGFDLAHAAGNIILQLHDWDVDCAVWCSYKYLNAGPGAAAGCFVHERYAQRPDLPRLAGWWGHNKDTRFQMPAGFDPIPGAEGWQISNPPIFQLAALKASMDIFDRAGMMRLRAKSERLTGYLEYLLRDRALPGVSLITPDDPAQRGAQLSLQIKQHGCALHQRLAEAHIICDWREPDVIRVAPVPLYNTFLDVLTFVNALDTAHREVLVSS

SEQ ID NO: 17 - protein, 424 aa, Candidatus Koribacter versatilis Ellin345
MAAAAFDTTENFAIEMDARDPMSRFRGRFHIPPAPDGSASVYLVGHSLGLQPKTVRAYLEQELKDWETLGVEGHFRGKHPWMPYHRLLTEQTARLVCAQPSEVVVMNSLTVNLHLMMVSFYRPTRERHNILIEGSAFPSDQYAVQSQIKFHGFDPASSLLELCPRVGEATMRDEDILELIEREGQSIALILLGGVNYATGQAFDMAEITKAGHAQGCVVAFDCAHAAGNLELKLHEWDVDWAAWCSYKYLNGGPGCIGGCFVHERYARDFELPRFAGWWGHDQETRFKMGPEFHPMAGAEGWQLSNPSILTMAALRASMEIFDEAGIGKLRQRSIALTGYLEFLLDQQKSARFEIITPREPERRGAQLSIRVAAGNRSVCDRLVEEGALCDWREPDILRVAPVPLYCSYRDCYRFVQRFVANLN

SEQ ID NO: 18 - protein, 428 aa, Cecembia lonarensis
MSNNQYEFSESFARQMDVQDTLSGFRDRFYFPQINGKEAIYFCGNSLGLQPKTVATYINKELDNWAKLGVDGHFYGEDAWYHVRKKSKPALSAIVGAHEHEVVAMNNLTSNLHFLMVSFYCPDQTRYKIITEAGAFPSDMYMLETQVKFHGLDPEKCIVELSPRAGEYTLRTEDILMAIEANKENLALVMMAGLQYYTGQVFDMKAITAAAHQVGARAGFDLAHAVGNAKLELHDWGVDFATWCSYKYLNSGPGNISGIFVHERHAENQELPRFAGWWGHDEGERFRMEKGFKPMYGADGWQLANSNVLALAAHQASLDIFEEAGMDRLRAKSELLTGYLEFLIEKISGDSGVLEIITPKIPNERGCQLSLLIHKGGKSVFDEFYKHGVVGDWRNPNVIRLAPTPLYNSFIDIYQFAKILEQSLQKFA

SEQ ID NO: 19 - protein, 421 aa, Chlamydia pecorum PV3056/3
MIEKLKQYHDEAISLDSLDPLQKFKECFTLPKEPGALYFCSNSLGLPAKAASQKLEEQLQRWSELGARGWFEGEGNWYNSLEESIVRPLSKILGAESNEVTLMNSLTVNLHMLLISFYRPTKTRYKILIDGPAFPSDLYAIKSHLRFHKKEEGLILIEPRPGEHLVQEEDFLRVIKIQGEEIALVFLNCVNFLSGQVLKVDEITRYAKEAGCCVGYDLAHAAGNIPLSLHDLGGDFAVGCSYKYLCGGPGGPGIAYVHASHHHQQFVRFSGWWGNDPNTRFYFPKEFVPYGGASSWQVSTPSILAKLPLIAALEVFEEAGMENIREKSKKQTAFLYTLLENARGTHFDMITPKEPELRGCQLSLRIKCSRSEEILRKLERLGITCDFRSPNILRVTPSPLYTSFYEIYRFAYTFLEVLKTI

SEQ ID NO: 20 - protein, 425 aa, Chlamydophila caviae GPIC
MNEILKHYQKKAAQLDEQDSLKHLRARFALPKDPNAIYFCNNSLGLPAVGAFTKIEELLQRWSDVGVNGWFEGVGNWYRSFDNPLRQPLSKILGAEYEEVVVMNSLTMNLHLLLVSFYRPTDTRYKILIEGPTFPSDLYAIKSQLSFHGKNPDDALIILEPRAGEDLLRYEDFQQTLEEQGESIALVFMNCVNFLTGQVLEVEAITNLAKEKGCVVGCDLAHAAGNIPLKLHEWGVDFALGCSYKYLCGGPGGPGIAFVHKSHHNEQLPRFSGWWGNDPETRFQMQLQPEFIPYSGAYSWQVSTPSIVSLMPLLATLEVFEEAGMERVRHKSKQMTAFLLELLELAPPSCFEIITPRDPELRGSQLSIRIQQHSEEVLQKLEAQRITCDSRPPDIIRVTATPLYNTFSEIYKFTCKLFEVLEIKS

SEQ ID NO: 21 - protein, 425 aa, Corallococcus coralloides DSM 2259
MTAPVYENTDVFAYGLDAADPLRPLRDEFLFPPAPSGAPAIYLAGNSLGLQPRKARKYVQMEMEDWERLGVEGHVHGRHPWLPYHEQLTDMVARVVGAQPIEVVVMNTLSVNLHLMMVSFYRPTRERFKILIEGGAFPSDQYAVASQARFHGYDPKEAIVRLMPREGEDTLRSEDILEAIERHGKELALVMLGSVNYLTGQAFDLREITRVAHAQGCKVGFDLAHAAGNLKLSLHDDGPDFAVWCSYKYLNGGPGSLGGVFVHERHAHSPQLPRFEGWWGHNKATRFEMGPTFDPLPGAEGWQLSNPPIFQLAALRSSLELFDKATMAALRTKSDQLTGYLEFLLDRLPAGYVSITTPRDLKQRGAQLSLRFKGEPKRLLQRLSAAGIICDFREPDIIRAAPTPLYNTYLDVFRFVKALEAHALE

SEQ ID NO: 22 - protein, 426 aa, Cyclobacterium marinum DSM 745
MDQIAFELTPEFARKMDLADPLSTYREKFYIPEKNGQPLIYFCGNSLGLQPRSVNAYLKQELEKWADKGVDGHFEGKVPWIDARKPSKRLIAPLVGANEQEVVAMNSLSVNLHLLMVSFYQPKGKKFKILTEAGAFPSDQYILESQVKFHGLLPDEAILEMAPRPNEHLLRTEDILQKIEDHKDELALIMLSGLQYYTGQLFDLEAISSAANKQGITIGFDLAHAIGNVPLRLHDWGVDFATWCSYKYLNSGPGNVSGIFVHEKHSDNALLPRFAGWWGHDEKERFKMKKGFKHMPGADGWLLSNDNVLGLAAHQASLELFAEAGLDKLRKKSIQLTNYLEFAIHETIKDSELLEIITPLKPTERGCQLSLLIHKKGKEVFDYWIDNGVVADWRNPNVIRLAPTPMYNTFQDVFEFSRILKNSLEA

SEQ ID NO: 23 - protein, 426 aa, Cystobacter fuscus
MSGEAVRFEPGEAFARRMDAEDPLRSFREEFLFPVHGDGHELYLLGNSLGLQPRKAKEYVLAAMEDWARLGVDGHFKGSPPWMEFHVGLGEQMARVVGARPEEVVVMNTLTVNLHLMMVSFYRPTPERSKILMEASAFPSDQYAVAAQVRHHGYSPEQTVIPLAPRPGEHTLRHEDILDTLERHGKEIALVLLGNVNYLTGQAFDMAAITRAAHQRGCRVGFDLAHAAGNLRLSLHEDGPDFAVWCTYKYLNGGPGALGGVFIHERHLRDASLHRLPGWWGNDRGTRFQMKPDFEPAPGAEGWVLSNPPIIQMAALRASLELFDRATMPALRAKSEKLTGYLEFLIDRLPEGFVHSLTPRDPGQRGAHLSLRFTKDPQRMLETLRAEGIHCDFRYPDIIRAAPVPLYNSFLDVHRFVSVLERYARG

SEQ ID NO: 24 - protein, 426 aa, Echinicola vietnamensis DSM 17526
MSSYRYSLAFAQERDREDPLRKFQSRFHFPKVNGEAAIYFCGNSLGLQPKAVREHLDRDLESWASKAVDGHFEGDAPWFSVHERSKAALAEIVGAKKHEVVAMGSLTTNLHALLVSFYQPNGKRNKILTEAGAFPSDMYALESQVKYHGLDPDEAIVEVGPRPGEHTIRTEDILQAISKHQDELACVMMAGLQYYTGQVFDMKAIASAAHAVGATVGFDLAHAAGNAPLHLHDWGVDFAAWCSYKYLNSGPGNVAGIFVHERHGNNPALNRFAGWWGHDEKVRFKMEKGFVPMYGADGWQNSNGNVLGMAAHQASLDIFQEAGMVHLRKKSVQLTGFLAFLIREISGESGVLEVITPNAEAERGCQLSLLIHKGGKAVFDEFYQNGIVGDWRNPNVIRIAPTPLYNSFEDVFRFAKILEQSLSKFA

SEQ ID NO: 25 - protein, 420 aa, Flavobacteria bacterium BBFL7
MEFNTTRDYALQLDQEDSLSRFRESFHIPKHTDGTDSIYLCGNSLGLQPRQTKTFLNQELDDWAKLGVEGHFHAENPWMPYHEFLTETTAQVVGAKPHEVVIMNTLTTNLHLMMVSFYQPKGKRTKIIIEADAFPSDRYAVASQVQFHGHDDKENIIEWAPRTGEHTPRLEDLETILKEQGDEIALIMVGAVNYYTGQFFDLKKITELGHAAGAMVGFDCAHGAGNVDLQLHDSGADFAVWCTYKYMNSGPGSLGGCFVHERHANNSELPRFTGWWGHNKDTRFKMRDDFEPMHGAEGWQLSNPPILSMVAIRASLDLFAQAGFENLRKKSIQLTNYLEYLVGELDGDRISIITPRDPKDRGCQLSLAVKNADKSLFDAITAKGVIADWREPDVIRIAPVPLYNNYEDCWRFVDVLKSEL

SEQ ID NO: 26 - protein, 442 aa, Flexibacter litoralis DSM 6794
MNFETTKNFASQLDNNDSLAHFRDKFWIPTLNSISKNTNSSNEKGKEKVVYFCGNSLGLQPKTTKAYIEQELEDWKNLGVEGHFHGKNPWLSYHKLLTNQTAKIVGAKPIEVVVMNNLTVNLHLLMVSFYRPNQKRFKILMEGGAFPSDQYAIESQVKFHGFSPDDAIVEMMPRKNENSEGEETLRTEDILKKIEELGDELALVMFGGVNYYTGQFFDLEKITQAAHKVGATAGFDLAHAAGNVPLKLHDWKVDFATWCSYKYLNSGAGGTSGVFINEKYADDDSLPRFAGWWGHDEKDRFKMKKGFIPMRGAEGWQLSNAQILPMAVHKASLDIFEEAGFENLRQKSEQLTVYMEFLIENFNKEQSKIKIKIITPKNKLERGCQLSLVFDKEGKKYHETLTKRGVISDWREPNVIRIAPIPLYNSFMDCYRFYEILKEIAV

SEQ ID NO: 27 - protein, 423 aa, Formosa sp. AK20
MSNYKPGLDYAKEQDQNDALSHYRSQFHIPKDNQGNNWLYFTGNSLGLQPKSTQKYIQQELDDWANLGVEGHFEAKNPWMPYHEFLTDSMAKIVGAKPIEVVTMNTLTTNLHLLMVSFYQPTKTKYKIVIESDAFPSDRYAVQTQLEFHGFDANEGLIEWKPRQGEELLNLDDLETILEEQGDEIALLLIGGVNYYTGQYLDLKKIAELGHAKNCMVGIDLAHGAGNIKPELHDSGVDFAAWCTYKYLNSGPGSLGGLFVHEKHAHNKKLKRFAGWWSHNKATRFNMRQPLDVIPGAEGWQLSNPPILSMAAIKASLDMFNEVGMDALREKSEKLTGYFEFLLNELNNDKVKIITPSNPKERGCQLSIQVRDADKSLHKKLTKAHIITDWREPDVIRCAPVPLYNSFEDVYRMVDKLKQILNT

SEQ ID NO: 28 - protein, 429 aa, Fulvivirga imtechensis
MAKDILHMTYENSLTFAQDLDRDDPLRHFRNKFHIPQLNDKDVIYFTGNSLGLQPKNTRVYIEEELEGWATLGVDGHFHSQKRPWFYYHKFSKEALAKIVGAKPSEVVSMNNLTVNLHLMMVSFYRPTSSRFKIMIEAGAFPSDQYAVESQIKFHGYNYEDALIEISPREGEYHLRTEDILSKIEENKDSLALVLFGGVQYYTGQLFDIGSITAAGHWAGAIVGFDLAHAAGNVPLNLHNDQVDFAAWCSYKYLNSGPGGVSGIFVHEKHGDAELPRFAGWWGHNESERFKMKKGFIPMSGADGWQLSNVNILSSAAHLAALEIYDEAGMEALRQKSIRLTGFMEYLLNGFNLGDDVLKIITPTDPAARGCQLSLLVSKNGKAIFEHLTRSGVVADWREPDVIRVAPVPLYNTFEDVYNFCEILKKVIF

SEQ ID NO: 29 - protein, 425 aa, Kangiella aquimarina
MTDIFSIDYARQLDQQDPISRMREQFHIPKQDNGDDEIYLCGNSLGLQPKRTQEYLNYELSQWQKLGVKGHFSGDFPWMPYHEFLTEESAKLVGAKNSEVVCMNSLTANLHFMMVSFYRPTATRNKILIEDHAFPSDHYAVESQVRYHGFDPDQAMLLAKPREGEETLRTEDLLNLIELHGEEIALIMLPGVQYYTGQVLDMKAITQAGHAKGCKVGFDLAHATGNIPMHLHDWDVDFAAWCSYKYLNSGPGSVAGCFVHEKHHTNMELPRFAGWWGHDKDSRFKMENHFIPMKSAEAWQLSNPPILSLAAIRASLDTIKDAGGIQALRDKSLKLSRYLRDLLEQELADEINILTPADEKASGCQLSLTVNLHGLDGKTVFDRIEAAGVTCDFRHPNVIRVAPVPLYNSFEDAYRFVTILKDSLK

SEQ ID NO: 30 - protein, 425 aa, Kangiella koreensis DSM 16069
MNNLFSLEHAQQLDQQDPLHHMRDQFHIPKQDNGDDEIYLCGNSLGLQPKRTQEYLNYELNQWQKLGVKGHFSGDFPWMPYHEFLTEESAKLVGAKNTEVVCMNSLTANLHFMMVSFYRPSKTRNKILIEDHAFPSDHYAVESQIRFHGFDPDQAMLLAKPREGEETLRTEDLLNLIEMHGDEIALIMLPGVQYYTGQVLDMKTITEAGHAKGCMVGFDLAHATGNIPMNLHDWNVDFAAWCTYKYLNSGPGSVAGCFVHEKHHSNLELPRFAGWWGHDKESRFRMENRFVPMQSAEAWQVSNPPILSLAAIRASLDTVKEAGGIDALREKSLKLTRYLRDLLEQELSEEINILTPADNSASGCQLSLTVNLHVLDGKTVFDRIEAAGVTCDFRHPNVIRVAPVPLYNSFEDAYRFVSILKDSLQ

SEQ ID NO: 31 - protein, 421 aa, Lacinutrix sp. 5H-3-7-4
MSNYTLGRDFAQQLDKEDQLAHYRNQFHIPKDKNGDDLIYLCGNSLGLQPKVTKDYINQELEDWANLGVEGHTEGKNPWLPYHEFLTESMAKVVGAKPIEVVVMNTLTANLHFMMVSFYKPTKKRYKILIEADAFPSDKYAVESQLRHHGFDDKEGLVLWKAREGEELANYEDLEAILEAQGDEIALIMIGGVNYYTGQFFDFKRIAALGHKNGCMVGFDCAHGAGNVNLDLHNSGADFAVWCTYKYMNAGPGSLSGCFVHERHAHNKDLNRFTGWWSHNKETRFNMRGEFDQLPGAEGWQLSNPPILSMAAIKASADIFAEVGMEKLTQKSKKLTGYFEFLLNELNNSDIKIITPSNPNERGCQLSIQVKNADKALHHKLTESGVISDWREPDVIRCAPVPLYNSFEDVYNMVERLKACL

SEQ ID NO: 32 - protein, 428 aa, Cecembia lonarensis
MTTTDFEYTEDFAKRMDDLDPFRHFRSMFHFPYVNGKEAIYFCGNSLGLQPKSVREYLDRELKNWELMAVDGHFHGEDAWYHVRKKSKPALAEIVGAHEHEVVAMNNLSSNLHFLMVSFYRPTKERYKIITEAGAFPSDMYMLETQVKFHGFDPADAIIEVAPRPGEYTIRTEDILAAIEDNQDELALVMMAGLQYYTGQVFDMEAITKAGHGIGVPVGFDLAHAAGNIPLRLHDWGVDFAAWCSYKYLNSGPGNISGIFVHERHADNTELPRFGGWWGHDEAIRFKMEKGFEPMYGADGWQLANSNVLALAVHQASLDIFQEAGMERLRTKSELLTGYLEFLIRKVGFANGVLEIITPNNPKERGCQLSLLVHKGGKLVFDHLYANGVVGDWRHPNVIRVAPTPLYNSFTDVFRFAKILEHSLQKFA

SEQ ID NO: 33 - protein, 429 aa, Mucilaginibacter paludis
MNYQNTLAFARELDEQDNLAGFRNEFIIPQHHGRDMIYLCGNSLGLQPKATAGVIAEQLSNWGSLAVEGWFEGDSPWMHYHKKLTEPLAAIVGALNTEVVAMNTLTVNLHFLLVSFYRPTAKKYKILMEGGAFPSDQYAIESQVHFHGYQPDDAIIEVFPRAGEDTLRTEDIIRTIHDHADDLALVLFGGINYYTGQFYDLEQITQAAHQVGAYAGFDLAHAAGNVPLQLHHWQVDFACWCSYKYMNSSPGGISGAFIHEKHFGNKELNRFAGWWGYREDKRFEMKPGFKPQEGAEGWQVSCSPLLLMAAHKASLNVFEKAGYIEPLRKKSKLLTGYLEYLIEGINTAHQKQLFKIITPKNENERGCQLSIVCDNGKAIFDQLVEGGVLGDWREPDVIRLSPIPLYNSFEDVYLAGKLLAGSVTQFFAE

SEQ ID NO: 34 - protein, 425 aa, Myroides odoratimimus
MSFENTLAYAKSLDEKDPLAKYRDEFNFPEVNGKQVIYFTGNSLGLQPKRAVEYVNEVMNDWGALAVEGHFYAEKPWWDYHERLSEPLSRIVGAKSSEITVMNTLTVNLHLLMTTFYRPTASKYKIICEEKAFPSDQYLIQSQVRLHGLDPKEAIIELKKRPGEHNFRLEDILEKIDEVGEEVALVLIGGLNYYTGQVFDIQTITAHAHQYGAKVGWDLAHAAGNIELKLHEWNVDFAAWCSYKYMNAGPGSASGCFIHERYHTDKDLVRLAGWWGHNKERRFLMEKKFDAVESAHGWQISNPSILSLAPYLASIEMFDEVGMEALITKQRKITAYLEFVMEDVAKAVNANYELITPKEESERGSQLSVFLHGKGKDLFSYLMNEGVIVDWREPNVVRLAPVPFYTSYEDIYRFGEILKKADSLF

SEQ ID NO: 35 - protein, 426 aa, Myxococcus fulvus HW-1
MTTPHAFEDTEAFAHTLDAEDALRGYRDAFHFPPGPDGKPVVYLAGNSLGLQPRNAARYIQEELEDWARLGVEGHHHGRHPWLHYHELVTEQAARLVGAKPLEVVVMNTLSVNLHLMMVSFYRPTKQRFKILVEAGAFPSDQYAVASQVRFHGHDAREAVLELKPREGEETLRTEDILDTLERHGHEVALVMLGSVNYLTGQAFDLAAITKAAHAKGCLVGFDLAHGAGNLKLSLHDDGPDFAVWCSYKYLNAGPGALGGVFVHERHAHTKDLPRFEGWWGHDKQTRFQMGPTFHALPGAEGWQLSNPPIFQLAALRASLELFDQAGMAALRAKSERLTGYLEFLLDKLPQGFVRITTPRDVKQRGAQLSLRFRGEPQGLLKRMGDAGIVCDFRKPDIIRAAPAPLYNSFTDVYRFVKALEGYARE

SEQ ID NO: 36 - protein, 425 aa, Myxococcus stipitatus DSM 14675
MTTHSFEDTEDFARRADEADALRSFRDAFHFPPGTDGKPLVYLAGNSLGLQPKNAARYVQEELEDWARFGVEGHHHGRHPWLHYHELVTEQAARLVGAKPQEVVVMNTLTVNLHLMMVSFYRPTKTRFKILVEGGAFPSDQYAVASQARFHGYDPREAILELKPRPGEETLRTEDILATLDQHGHEVALVMLGSVNYLTGQAFDIPAITKTAHAKGCFVGFDLAHGAGNLKLALHDDGPDFAVWCSYKYLNGGPGALAGVFVHERHARSKDIPRFEGWWGHDKATRFQMGPTFDPLPGAEGWQLSNPPILQLAALRASFELFDQAGMEALRAKSEKLTGYLEFLLEKLPPGFVRIITPRDVKQRGAQLSLRFKGEAQGMLKRLSDAGIICDFRKPDIIRAAPAPLYCSFTDVYRFVRTLEAHARD

SEQ ID NO: 37 - protein, 426 aa, Myxococcus xanthus DK 1622
MTTPYLFEDSESFARKLDAEDALRGYRDAFHFPPGPDGKPVVYLAGNSLGLQPRNAARYIQEELEDWARLGVEGHHHGRHPWLHYHELVTEHAARLVGAKPLEVVVMNTLSVNLHLMMVSFYRPTKQRFKILVEAGAFPSDQYAVASQVRFHGYDAREAVLELKPREGEETLRTEDILETIERHGHEVALVMLGSVNYLTGQAFDLAAITKAAHAKGCFVGFDLAHGAGNLRLSLHDDGPDFAVWCSYKYLNAGPGALGGVFVHERHAHTKDLPRFEGWWGHDKQTRFQMGPTFSALPGAEGWQLSNPPIFQLAALRASLELFDQAGMAALRAKSERLTGYLEFLLDRLPEGFVRITTPRDVKQRGAQLSLRFRGEPQGLLKRLGDAGIICDFRKPDIIRAAPAPLYNSFTDVYRFVKTLEGHARE

SEQ ID NO: 38 - protein, 428 aa, Nafulsella turpanensis
MINQYQSNQAYAREQDARDPLRQFREQFIIPPAKSGGEAIYFCGNSLGLQPKNTRSYLDRELEKWATYAVDGHFHAPEPWLHYHRLLKEPLARIVGAKPEEVVVMNNLSSNLHFLMVSFYQPTTKRYKVLMEGGAFPSDQYAVESQVKFRGYTPEEAIVEVFPREGEQTLRTEDILAAIEQHQDELALVLFAGLQYYTGQVFDMAAITKAGQAAGAKVGFDLAHAAGNVPLQLHDWGVDFAAWCSYKYLNSGPGSNSGIFVHERYANQAELPRFAGWWGHDEKERFLMQKGFKPMYGADGWQLSNGNILPLAAQRASLEIFEQAGMDNLRQKSIQLTGYLEYLIREEVSSKANRLQIITPSQPEERGCQLSLFVEKNGKQLFEQISQAGVVGDWREPNVIRVAPTPLYNTFTDVFQFAQLLKKAIKEQ

SEQ ID NO: 39 - protein, 428 aa, Niastella koreensis GR20-10
MIFENSHSFAYVLDEQDELRSFREQFIMPVIDGKQQIYFLGNSLGLQPKRTNDYLQQVLNKWANYGVEGFFMGEQPWLQYHDHLTKPLSTIVGALPHEVVAMNQLTVNLHLLLVSFYNPHGKRNKIICEAKAFPSDQYMLETHVKYCGFNPDDVIVEVGPRKGEHTIRHEDILQAIQQHKDELALVLWGGMNYYTGQLFDMAAITKAAQAVGAKVGFDLAHAAGNVPLQLHNWNVDFAAWCSYKYMNSGPGGIGGAYIHERYHNDTSLPRFAGWWGYDKATRFLMQKGFNATRSAEGWQLSTPSPLLYAAHRAALDLFMEAGFNRLQNKRQLLNKWLWFLLDDLNNAQTEPVVEFITPRNEAERGCQVSMLMLQQGKQVFDELARAGVIVDWREPNVIRLAPVPLYNSFEEVWQFTNILRQILQLQHA

SEQ ID NO: 40 - protein, 420 aa, Nonlabens dokdonensis DSW-6
MNFKTDHNFAIELNKSDSLSRFRESFHIPKHTDGTDSIYLCGNSLGLQPRQTKTFLNQELDDWARLGVEGHFHAAHPWMPYHEFLTETTAQIVGAKPHEVVIMNTLTTNLHLMMVSFYQPKGKRTKIIIEADAFPSDRYAVASQVKFHGHDDKENIIEWSPRAGEHTPRIEDLENLLKEQGDEIALIMVGAVNYYTGQFFDLKKITELGHAAGAMVGFDCAHGAGNVDLQLHNSGADFAVWCTYKYMNSGPGSLGGCFVHERHASNSDLPRFTGWWGHNKDTRFKMRDDFEPMHGAEGWQLSNPPILSMVAIRASLDLFAQAGFENLRQKSIQLTNYLEYLLSNLEGDRISIITPENPKDRGCQLSLAVKNADKSLFDAITEKGVIADWREPDVIRIAPVPLYNNYEDCWRFVDVLKSEL

SEQ ID NO: 41 - protein, 431 aa, Pedobacter agri
MKLENTLAFAKEQDEKDELKHFRDQFLFPKYQDKFFIYLCGNSLGLQPKVAKEVINSQLDNWANLAVEGWFDGEEPWMYYHKELKKLMAPIVGALPSEVCPMNTLTVNLHLLMISFYQPQGKRFKIIMEGGAFPSDQYAIESQVRFHGFDPSDAIIEVFPREGEEILRTEDIVAKIKEHGDEIALLLFGGINYYTGQWYDMENITKAGHSIGAMVGWDLAHAAGNVPVKLHDWNVDFACWCSYKYQNAGPGGISGIFVHEKHFENKALNRFAGWWGYQENKRFKMEKGFVPEAGADGWQVSCTQVMPMALYHASLQIFKEAGFLNTLRNKSISLTSYLEFVVNELNIELEKEQYKIITPKNSAERGAQLSIIAARNGKEIFDGLLAHGILGDWREPNVIRLSPVPLYNSFEDIYQTGKALSEVTRKILTTA

SEQ ID NO: 42 - protein, 449 aa, Pedobacter sp. BAL39
MKVVDNKKTGLFNYIPFLWIFGTMNFENTLAFAQGLDQADPLRDLRNEFLFPQQNGKPFIYLCGNSLGLQPKVAREVLDRQLNNWQNLAVEGWFEGETPWMYYHKALKELMAPIVGARPAEVCPMNTLTVNLHLLMVSFYKPKAKRFKIMMEAGAFPSDQYAIESQVRFHGYDPKDAIIEVSPRPGEYTLRTEDILEQISLQGDQIALVLFGGINYFTGQWFDMEAITRAGHQAGAVVGFDLAHAAGNVPVQLHDWDVDFACWCSYKYQNSGPGGISGIFVHERHFGDQTLSRFAGWWGYQESQRFKMEKGFVPEAGADGWQVSCTQVMPMALYHAALQIFEKAGFIGPLRKKSKALTAYLFYLINEVNNELCEMQYQVITPSSAEDRGAQVSIIAKANGKYIFEQLVANNVLGDWREPNVIRLSPVPSYNSFEDVFRTAELLLQIGRK

SEQ ID NO: 43 - protein, 428 aa, Pedobacter sp. V48
MNFENNLAFAQSLDQADPLSSFRHDFLFPQQNGNPFIYLCGNSLGLQPKAVRKVVDEQLNNWRNLAVEGWFEGDNPWMFYHKELKKLMGPLVGASTDEVCPMNTLTVNLHLLMVSFYKPVRGRFKIIMEAGAFPSDQYAVESQVRFHGYDAKEAIVEVAPRIGEYILRTEDILAQIAKHGDEVALVLFSGVNYFTGQWFDMEAITMAGHAEGAVVGFDLAHAAGNVPLKLHDWDIDFACWCSYKYQNSGPGGISGIFVHEKHFTDTTLNRFAGWWGYQQAHRFKMEKGFLPEPGADGWQVSCTQVMPMALYFASLQIFEKAGFIEPLRLKSKTLTSYLFHIVNQVNKLLSCEQFEIITPDNENERGAQVSIIAKQKGKEIFEKLIANNVLGDWREPNVIRLSPVPLYNSFEDVFRTGELLLQITKGVI

SEQ ID NO: 44 - protein, 428 aa, Rhodonellum psychrophilum
MKDIKYEYSEFFARQLDNEDPLKDFRNEFYFPKIEGKEAIYFCGNSLGLQPRSTKEYIQRELDNWAELAVDGHFKGEDAWYHVRKKSKPALSEIVGAHEHEVVAMNNLSSNLHFLMVSFYRPSKTRFKIITEAGAFPSDMYMLETQVKFHGLDPEKTIIEVAPRPGEHTLRTEDILLAIEEQGEELALVMMAGLQYYTGQVFDMESITRAGHSVGANVGFDLAHAAGNVPMSLHDWGVDFATWCSYKYMNSGPGNVSGVFVHERHAQNPDLPRFAGWWGHDEEERFKMEKGFKPMYGADGWQVANSNVLALAAHQSSLDIFERAGIKNLREKSELLTGYLEFLIQQISGDSGVIEIITPKNPQERGCQLSLLVHKGGKAVFDELYLNGIIGDWRHPKVMRIAPTPLHNSFLDVFRFAQILEKSILKFA

SEQ ID NO: 45 - protein, 430 aa, Salinispora arenicola
MNKEELDQEEKAANRLDTADPGHRHLFHLPPSDGGRYQQAAYLAGNSLGLQPLATRDELLADLDAWRRLGVEGHLEADRPWLPYHELLTAPTARLVGARPAEVVVMNSLTVNLHLLMVSFYRPVGARTRIVIEDNAFPSDSYAVRSQARFHGLDPDTTVVRLAPRPGEDTLRTVDVLDLLAAEGDTIALVLLGGVNYLTGELLDIPAITAAGRAAGAAVGWDLAHAAGNVPLSLHDWDVDFAAWCSYKYLNSGPGGLSSVFVHERHLADPTLPRFEGWWSTDAAVRFEMSPVARPPATAEAWQVSNPPIFAMGPVRTSLELFDSVGMTALRERSVRLTGYLEWLLDQITPGRQLAVVTPRDPDRRGAQLSVRVGSGSAAELTKRLRCEYGVIADAREPDIVRFAPVPLYSTYHDCWRVADALAATVEVRG

SEQ ID NO: 46 - protein, 425 aa, Saprospira grandis str. Lewin
MQEVQFEDALDYAKAQDVSDPLAHFRPQFHFPKQADGSPIIYLCGNSLGLQPRLAQQLMQDEMDVWKELAVEGHFKAERPWMTYHEEFSRQLSPIVGALPKEITVMNTLSVNLHLMMVSFYRPTKSRYKIVIEGGAFPSDKYAVDSQLRFHGIDPQDGLIQLRPRMGEDHLRTEDILQALEREKDSIALVMLSGINYYTGQCFDMKSITKKGHEIGAMVGFDLAHAAGNVRLQLHDWGMDFAVWCHYKYLNSGPGCIAGAFVHERHLNRKDLPRFEGWWGHHKESRFKMPATFEPAPNADAWQISNAPILAMVPMRASLALFNEAGMDRLLAKSKKLTAYLEFLLNQLPTDRIRILTPKDPKDRGAQLSIQVKGADRSLFDDLVKNGVIGDWREPDVIRISPAPIYNSFEDVYRMVQILKKCLQL

SEQ ID NO: 47 - protein, 427 aa, Stigmatella aurantiaca DW4/3-1
MTEASMRFEEGEGFARRMDAEDPLRSFREEFLFPQSPQGEPLVYLAGNSLGLQPRRAQQYVQEEMEDWARLGVEGHFHARRPWLPYHENLTGQTARLVGALPLEVVVMNTLSVNLHLMMVSFYRPTRERFKILIEGGAFPSDQYAVASQARFHGFDPKDAVLKLEPRAGEDTLRTEDILETLERHGSEIALVLLGNVNYLTGQAFDMKALTQAAHARGCRVGFDLAHGAGNLRLSLHDDGPDFAVWCSYKYLNGGPGALGGVFIHERHARAEGLPRFEGWWGNDKAIRFQMGPDFVPLPGAEGWQLSNPPIFQLAALRASMELFDRATMPSLRGKGDRLTGYLEFLLDRLPSGFVRITTPRDVKARGSQLSLRFSKDPRRLLTRLSEAGVCCDFRSPDIIRAAPAPLYNSFQDVYRFVKVLESHARD

SEQ ID NO: 48 - protein, 423 aa, Xanthomonas axonopodis
MTDPLSRAHAAALDAADPLRNLRDAFVFPQHGDDDQTYFVGNSLGLQPRAARAMVDEVLDQWGALAVEGHFTGPTQWLTYHQLVRDALARVVGAQPGEVVAMNTLSVNLHLMMASFYRPTAERGAILIEAGAFPSDRHAVESQLRLHGLDPATHLIEVEADEPNGTVSMSAIAEAIAQHGPHLALVLWPGIQYRTGQAFDLAEIVRLARAQGAAVGFDLAHAVGNLPLTLHDDGVDFAVWCHYKYLNAGPGAVGGCFVHARHATSDLPRMAGWWGHEQQTRFRMDPQFVPSPGAEGWQLSNPPVLALAPLRASLALFDQAGMAALRAKSEQLTGHLEQLIHARAPQVLQIVTPVEPARRGCQLSLRVAGGRARGRALFEHLHAAGVLGDWREPDVIRIAPVPLYNRFSDLHTFVEQVEAWAAA

SEQ ID NO: 49 - protein, 422 aa, Psychroflexus gondwanensis
MKYQNTKSFAEQLDEADPLKAYRSEFLFPKAKDGSPKVYLCGNSLGLQPKQTSAFIQQELQDWADLGVEGHSHATHPWMTSNEDLADSMAKIVGAQPQEVVIMNTLTVNLHLMMVSFYKPTPKKFKILIESDAFPSDKYAVESQLKFHNIDPKEGLLLWKPRPGEHLCRTEDFEQIIEEHGDEIALVMIGSTNYYSGQAYDLKRITEVSKTKDITVGFDLAHGAGNIQPNLHDIGADFAVWCTYKYLNSGPGSLGGCFIHEKHIADEHINRFVGWWGHNKDSRFNMRVDFDPIPTADGWQLSNPPILSLAGTRSSLDLFDKAGFDNIRKKSVLLTGFLEFLIDDLDMEEISILTPRSPEERGCQLSIQVKNANKSLFHQLMDKGVVADWREPDVIRIAPAPLYNSYTDVFTFVEILKHCLNA

SEQ ID NO: 50 - protein, 422 aa, Lewinella cohaerens
MTYQATREYAQSQDDKDPMRGFRERFHLPRQANGEPFIYLCGNSLGLQPKSTKAAIDQELLDWQNLGVEGHLHAKNPWLPYHEFLTEKMAEIVGAKPIEVVMMNTLTVNLHLMMVSFYRPEGKRTKILMEADAFPSDRYAISSQLKFHGYDPAEHLVELKARDGEVLIREEDIAHILEEQGAEIALVLLGNTNYYTGQFFNMPEITKLAHAQGCMVGFDCAHGAGNVPLDLHDSGADFAVWCSYKYINSGPGSVSGCFVHERHAHDKELPRFTGWWGHNKVTRFGMRDDFDPIPGVEAWQLSNPPILSLAAIKASLEVFAEAGMNNLRQKSLALTGYLEYLVDQLPGGKISIITPRDPERRGCQLSIQVQDADKSLYEAISAAGVIADWREPDVIRVAPVPLYNTFTEVYDFVKILGEKMEA

SEQ ID NO: 51 - protein, 425 aa, Lewinella persica
MVEEFQNDLAFARKMDERDELRAYRSQYHMPVQANGQPYVYLCGNSLGLQPKATEGYLLQELEDWKNLGVEGHFHAKNPWMPYHEFLTEAMARVVGAKPSEVVVMNTLTVNLHLMMVSFYRPVGRRKKIIIEADAFPSDKYAVESQIRFHGLSPEDCLIELKARDGEVCLRQEDILGVIDAHSEDIALILLGNTNYYTGQFFDMKTISEHGHAKGCMVGFDCAHGAGNVPLNLHDSGCDFAVWCNYKYLNSGPGGMGGAFIHERHADSKDIPRFEGWWGHNKETRFKMRDAFDPTPGTEAWQLSNPPILAMVAVWSALKLFDEVGMTRLRKKAISLTGYLEYLVNTLGDDVVNIVTPADPAQRGSQLSIQVKTADKKLFNKITEAGVIADWREPDVIRVAPVPMYNSYEDVYNFYTILKSAIAGN

SEQ ID NO: 52 - protein, 424 aa, Pontibacter roseus
MNYQNTLAFAQEQDNLDPLKHFKDRFYFPQVNGRDAIYFCGNSLGLQPKSAQMYIDNEMYKWANYAVEGHFKVEEPWFNYHRLLTDGAARVVGARPQEVVIMNQLTVNLHLMLVSFYRPEGRRIKIIMEGGAFPSDQYALETQVKFHGYTPEEAIIELFPREGEHTLRTEDILKSIEAAGDELALVLMGGINYYTGQVYDMAAITQAGHGVGAVVGFDLAHAAGNVPLQLHDWGVDFAVWCTYKYLNSGPGGTAGVFVHERHANNPDLPRFAGWWGHDASVRFQMKKGFIPMTGAEGWQLSNAQILPMAVHRAALELFDEAGMDNLRAKSEKLTGYLEYLIDDVHVGKELLEMITPRDPQARGCQISLLVKQNARELFNRLMEAGIIVDFREPSVIRVAPTPLYNSFEEVYRFSEILHDCLQSH

SEQ ID NO: 53 - DNA, 1304 bp, Artificial Sequence
  Synthetic polynucleotide
ccatgggcggacaccatcatcaccaccacggcggcattgaaaaactgaaacagtatcacgatgaagcgatcagcctggatagccttgatcccttacagaaattcaaagaatgctttacattaccgaaggaacctggagcactgtatttctgcagcaatagtctgggcttgcccgcgaaagcggcttcccagaaactggaagaacagttacagcggtggagcgaattaggcgctcgtggatggtttgaaggcgagggtaattggtataacagcttggaagagcctattgtgcgtccattgagcaaaatcttaggagcggaaagcaatgaagtgaccctgatgaatagcttgaccgtgaatctgcacatgttgttgattagtttctatcgtccgaccaaaatgcgttataagatactgattgatggcccagcctttccgtccgatctgtatgccattaagtcgcatctgcgttttcataagaaagaagaaggtcttattctgatagaaccgcgtccgggcgaacatctggtgcaggaagaagactttctgcgcgtgataaagaagcaaggagaggaaattgcgttggtgtttctgaactgcgtgaattttctgagcggccaggtgctgaaagtggatgaaatcacccgttatgccaaggaggctggctgctgcgtcggttatgatctggcgcatgcagcaggcaatattcccttaagcttgcatgatcttggcggcgactttgcggtgggctgctcctacaaatatctgtgcggaggcccaggaggtccaggcatagcctacgttcacgcgtcacatcaccaccaacagttcgtgcgtttcagcgggtggtggggcaatgatccgaatacccggttttacttccccaaagagtttgtgccgtatggcggtgcgagctcctggcaggtgagcaccccgtcgattctggcgaaactgccgttaattgcggcactggaggtgtttgaggaagcgggcatggagaatatacgtgaaaagagcaagaaacaaacagcgttcctgtataccctgttagaaaatgctcgcggcacccattttgatatgataaccccgaaagaaccggagctgcgtggctgtcagcttagcctgcgtatcaaatgcagccgtagcgaagagatcttacggaagctggaacgtttaggcattacatgcgatttccgttcgccgaacattctgcgtgtggcgccgagcccgttgtacaccagcttttacgaaatctatcgttttgcgtacacctttctggaagtcctgaaaaccatttgagaattc

SEQ ID NO: 54 - protein, 431 aa, Artificial Sequence
  Synthetic polypeptide
MGGHHHHHHGGIEKLKQYHDEAISLDSLDPLQKFKECFTLPKEPGALYFCSNSLGLPAKAASQKLEEQLQRWSELGARGWFEGEGNWYNSLEEPIVRPLSKILGAESNEVTLMNSLTVNLHMLLISFYRPTKMRYKILIDGPAFPSDLYAIKSHLRFHKKEEGLILIEPRPGEHLVQEEDFLRVIKKQGEEIALVFLNCVNFLSGQVLKVDEITRYAKEAGCCVGYDLAHAAGNIPLSLHDLGGDFAVGCSYKYLCGGPGGPGIAYVHASHHHQQFVRFSGWWGNDPNTRFYFPKEFVPYGGASSWQVSTPSILAKLPLIAALEVFEEAGMENIREKSKKQTAFLYTLLENARGTHFDMITPKEPELRGCQLSLRIKCSRSEEILRKLERLGITCDFRSPNILRVAPSPLYTSFYEIYRFAYTFLEVLKTI

SEQ ID NO: 55 - protein, 465 aa, Artificial Sequence
  Synthetic polypeptide
MEPSSLELPADTVQRIAAELKCHPTDERVALHLDEEDKLRHFRECFYIPKIQDLPPVDLSLVNKDENAIYFLGNSLGLQPKMVKTYLEEELDKWAKIAAYGHEVGKRPWITGDESIVGLMKDIVGANEKEIALMNALTVNLHLLMLSFFKPTPKRYKILLEAKAFPSDHYAIESQLQLHGLNIEESMRMIKPREGEETLRIEDILEVIEKEGDSIAVILFSGVHFYTGQHFNIPAITKAGQAKGCYVGFDLAHAVGNVELYLHDWGVDFACWCSYKYLNAGAGGIAGAFIHEKHAHTIKPALVGWMGHELSTRFKMDNKLQLIPGVCGFRISNPPILLVCSLHASLEIFKQATMKALRKKSVLLTGYLEYLIKHNYGKDKAATKKPVVNIITPSHVEERGCQLTITFSVPNKDVFQELEKRGVVCDKRNPNGIRVAPVPLYNSFHDVYKFTNLLTSILDSAETKN

SEQ ID NO: 56 - protein, 465 aa, Artificial Sequence
  Synthetic polypeptide
MEPSSLELPADTVQRIAAELKCHPTDERVALHLDEEDKLRHFRECFYIPKIQDLPPVDLSLVNKDENAIYFLGNSLGLQPKMVKTYLEEELDKWAKIAAYGHEVGKRPWITGDESIVGLMKDIVGANEKEIALMNALTVNLHLLMLSFFKPTPKRYKILLEAKAFPSDHYAIESQLQLHGLNIEESMRMIKPREGEETLRIEDILEVIEKEGDSIAVILFSGVHFYTGQHFNIPAITKAGQAKGCYVGFDLAHAVGNVELYLHDWGVDFACWCSYKYLNAGAGGIAGAFIHEKHAHTIKPALVGWLGHELSTRFKMDNKLQLIPGVCGFRISNPPILLVCSLHASLEIFKQATMKALRKKSVLLTGYLEYLIKHNYGKDKAATKKPVVNIITPSHVEERGCQLTITFSVPNKDVFQELEKRGVVCDKRNPNGIRVAPVPLYNSFHDVYKFTNLLTSILDSAETKN

SEQ ID NO: 57 - protein, 420 aa, Chlamydophila pecorum
IEKLKQYHDEAISLDSLDPLQKFKECFTLPKEPGALYFCSNSLGLPAKAASQKLEEQLQRWSELGARGWFEGEGNWYNSLEEPIVRPLSKILGAESNEVTLMNSLTVNLHMLLISFYRPTKMRYKILIDGPAFPSDLYAIKSHLRFHKKEEGLILIEPRPGEHLVQEEDFLRVIKKQGEEIALVFLNCVNFLSGQVLKVDEITRYAKEAGCCVGYDLAHAAGNIPLSLHDLGGDFAVGCSYKYLCGGPGGPGIAYVHASHHHQQFVRFSGWWGNDPNTRFYFPKEFVPYGGASSWQVSTPSILAKLPLIAALEVFEEAGMENIREKSKKQTAFLYTLLENARGTHFDMITPKEPELRGCQLSLRIKCSRSEEILRKLERLGITCDFRSPNILRVAPSPLYTSFYEIYRFAYTFLEVLKTI

SEQ ID NO: 58 - protein, 465 aa, Artificial Sequence
  Synthetic polypeptide
MEPSSLELPADTVQRIAAELKCHPTDERVALHLDEEDKLRHFRECFYIPKIQDLPPVDLSLVNKDENAIYFLGNSLGLQPKMVKTYLEEELDKWAKIAAYGHEVGKRPWITGDESIVGLMKDIVGANEKEIALMNALTVNLHLLMLSFFKPTPKRYKILLEAKAFPSDHYAIESQLQLHGLNIEESMRMIKPREGEETLRIEDILEVIEKEGDSIAVILFSGVHFYTGQHFNIPAITKAGQAKGCYVGFDLAHAVGNVELYLHDWGVDFACWCSYKYLNAGAGGIAGAFIHEKHAHTIKPALVGWFGHELSTRFKMDNKLQLIPGVCGFRISNPPILLVCSLHASLEIFKQATMKALRKKSVLLTGYLEYLIKHNYGKDKAATKKPVVNIITPSHVEERGCQLTITFSVPNKDVFQELEKRGVVCDKRNPNGIRVTPVPLYNSFHDVYKFTNLLTSILDSAETKN

SEQ ID NO: 59 - protein, 465 aa, Artificial Sequence
  Synthetic polypeptide
MEPSSLELPADTVQRIAAELKCHPTDERVALHLDEEDKLRHFRECFYIPKIQDLPPVDLSLVNKDENAIYFLGNSLGLQPKMVKTYLEEELDKWAKIAFYGHEVGKRPWITADESIVGLMKDIVGANEKEIALMNALTVNLHLLMLSFFKPTPKRYKILLEAKAFPSDHYAIESQLQLHGLNIEESMRMIKPREGEETLRIEDILEVIEKEGDSIAVILFSGVHFYTGQHFNIPAITKAGQAKGCYVGFDLAHAVGNVELYLHDWGVDFACWCSYKYLNAGAGGIAGAFIHEKHAHTIKPALVGWYGHELSTRFKMDNKLQLIPGVCGFRISNPPILLACSLHASLEIFKQATMKALRKKSVLLTGYLEYLIKHNYGKDKAATKKPVVNIITPSHVEERGCQLTLTFNVPNKDVFQELEKRGVVCDKRNPNGIRVAPVPLYNSFHDVYKFTNLLTSILDSAETKN

SEQ ID NO: 60 - protein, 465 aa, Artificial Sequence
  Synthetic polypeptide
MEPSSLELPADTVQRIAAELKCHPTDERVALHLDEEDKLRHFRECFYIPKIQDLPPVDLSLVNKDENAIYFLGNSLGLQPKMVKTYLEEELDKWAKIAIYGHEVGKRPWITGDESIVGLMKDIVGANEKEVALMNALTVNLHLLMLSFFKPTPKRYKILLEAKAFPSDHYAIESQLQLHGLNIEESMRMIKPREGEETLRIEDILEVIEKEGDSIAVILFSGVHFYTGQHFNIPAITKAGQAKGCYVGWDLAHAVGNVELYLHDWGVDFACWCSYKYLNAGAGGIAGAFIHEKHAHTIKPALVGWFGHELSTRFKMDNKLQLIPGVCGFRISNPPILLVCSLHASLEIFKQATMKALRKKSVLLTGYLEYLIKHNYGKDKAATKKPVVNIITPSHVEERGCQLTITFSVPNKDVFQELEKRGVVCDKRNPNGIRVAPVPLYNSFHDVYKFTNLLTSILDSAETKN

SEQ ID NO: 61 - protein, 465 aa, Artificial Sequence
  Synthetic polypeptide
MEPSSLELPADTVQRIAAELKCHPTDERVALHLDEEDKLRHFRECFYIPKIQDLPPVDLSLVNKDENAIYFLGNSLGLQPKMVKTYLEEELDKWAKIAIYGHEVGKRPWITGDESIVGLMKDIVGANEKEVALMNALTVNLHLLMLSFFKPTPKRYKILLEAKAFPSDHYAIESQLQLHGLNIEESMRMIKPREGEETLRIEDILEVIEKEGDSIAVILFSGVHFYTGQHFNIPAITKAGQAKGCYVGWDLAHAVGNVPLYLHDWGVDFACWCSYKYLNAGAGGIAGAFIHEKHAHTIKPALVGWFGHELSTRFKMDNKLQLIPGVCGFRISNPPILLVCSLHASLEIFKQATMKALRKKSVLLTGYLEYLIKHNYGKDKAATKKPVVNIITPSHVEERGCQLTITFSVPNKDVFQELEKRGVVCDKRNPNGIRVAPVPLYNSFHDVYKFTNLLTSILDSAETKN

SEQ ID NO: 62 - protein, 465 aa, Artificial Sequence
  Synthetic polypeptide
MEPSSLELPADTVQRIAAELKCHPTDERVALHLDEEDKLRHFRECFYIPKIQDLPPVDLSLVNKDENAIYFLGNSLGLQPKMVKTYLEEELDKWAKIAIYGHEVGKRPWITGDESIVGLMKDIVGANEKEVALMNALTVNLHLLMLSFFKPTPKRYKILLEAKAFPSDHYAIESQLQLHGLNIEESMRMIKPREGEETLRIEDILEVIEKEGDSIAVILFSGVHFYTGQHFNIPAITKAGQAKGCYVGWDLAHAVGNVPLYLHDWGVDFACWCSYKYLNAGAGGIAGAFIHEKHAHTIKPALVGWLGHELSTRFKMDNKLQLIPGVCGFRISNPPILLVCSLHASLEIFKQATMKALRKKSVLLTGYLEYLIKHNYGKDKAATKKPVVNIITPSHVEERGCQLTITFSVPNKDVFQELEKRGVVCDKRNPNGIRVAPVPLYNSFHDVYKFTNLLTSILDSAETKN

SEQ ID NO: 63 - protein, 465 aa, Artificial Sequence
  Synthetic polypeptide
MEPSSLELPADTVQRIAAELKCHPTDERVALHLDEEDKLRHFRECFYIPKIQDLPPVDLSLVNKDENAIYFLGNSLGLQPKMVKTYLEEELDKWAKIASYGHEVGKRPWITGDESIVGLMKDIVGANEKEIALMNALTVNLHLLMLSFFKPTPKRYKILLEAKAFPSDHYAIESQLQLHGLNIEESMRMIKPREGEETLRIEDILEVIEKEGDSIAVILFSGVHFYTGQHFNIPAITKAGQAKGCYVGFDLAHAVGNVELYLHDWGVDFACWCSYKYLNAGAGGIAGAFIHEKHAHTIKPALVGWLGHELSTRFKMDNKLQLIPGVCGFRISNPPILLVCSLHASLEIFKQATMKALRKKSVLLTGYLEYLIKHNYGKDKAATKKPVVNIITPSHVEERGCQLTITFSVPNKDVFQELEKRGVVCDKRNPNGIRVAPVPLYNSFHDVYKFTNLLTSILDSAETKN

SEQ ID NO: 64 - protein, 465 aa, Artificial Sequence
  Synthetic polypeptide
MEPSSLELPADTVQRIAAELKCHPTDERVALHLDEEDKLRHFRECFYIPKIQDLPPVDLSLVNKDENAIYFLGNSLGLQPKMVKTYLEEELDKWAKIASYGHEVGKRPWITGDESIVGLMKDIVGANEKEIALMNALTVNLHLLMLSFFKPTPKRYKILLEAKAFPSDHYAIESQLQLHGLNIEESMRMIKPREGEETLRIEDILEVIEKEGDSIAVILFSGVHFYTGQHFNIPAITKAGQAKGCYVGFDLAHAVGNVELYLHDWGVDFACWCSYKYLNAGAGGIAGAFIHEKHAHTIKPALVGWLGHELSTRFKMDNKLQLIPGVCGFRISNPPILLVCSLHASLEIFKQATMKALRKKSVLLTGYLEYLIKHNYGKDKAATKKPVVNIITPSHVEERGCQLTITFSVPNKDVFQELEKRGVVCDKRNPNGIRVTPVPLYNSFHDVYKFTNLLTSILDSAETKN

SEQ ID NO: 65 - protein, 465 aa, Artificial Sequence
  Synthetic polypeptide
MEPSSLELPADTVQRIAAELKCHPTDERVALHLDEEDKLRHFRECFYIPKIQDLPPVDLSLVNKDENAIYFLGNSLGLQPKMVKTYLEEELDKWAKIASYGHEVGKRPWITGDESIVGLMKDIVGANEKEIALMNALSVNLHLLMLSFFKPTPKRYKILLEAKAFPSDHYAIESQLQLHGLNIEESMRMIKPREGEETLRIEDILEVIEKEGDSIAVILFSGVHFYTGQHFNIPAITKAGQAKGCYVGFDLAHAVGNVELYLHDWGVDFACWCSYKYLNAGAGGIAGAFIHEKHAHTIKPALVGWLGHELSTRFKMDNKLQLIPGVCGFRISNPPILLVCSLHASLEIFKQATMKALRKKSVLLTGYLEYLIKHNYGKDKAATKKPVVNIITPSHVEERGCQLTITFSVPNKDVFQELEKRGVVCDKRNPNGIRVTPVPLYNSFHDVYKFTNLLTSILDSAETKN

SEQ ID NO: 66 - protein, 465 aa, Artificial Sequence
  Synthetic polypeptide
MEPSSLELPADTVQRIAAELKCHPTDERVALHLDEEDKLRHFRECFYIPKIQDLPPVDLSLVNKDENAIYFLGNSLGLQPKMVKTYLEEELDKWAKIAVYGHEVGKRPWITADESIVGLMKDIVGANEKEIALMNALTVNLHLLMLSFFKPTPKRYKILLEAKAFPSDHYAIESQLQLHGLNIEESMRMIKPREGEETLRIEDILEVIEKEGDSIAVILFSGVHFYTGQHFNIPAITKAGQAKGCYVGFDLAHAVGNVELYLHDWGVDFACWCSYKYLNAGAGGIAGAFIHEKHAHTIKPALVGWYGHELSTRFKMDNKLQLIPGVCGFRISNPPIVLVCSLHASLEIFKQATMKALRKKSVLLTGYLEYLIKHNYGKDKAATKKPVVNIITPSHVEERGCQLTLTFNVPNKDVFQELEKRGVVCDKRNPNGIRVAPVPLYNSFHDVYKFTNLLTSILDSAETKN

SEQ ID NO: 67 - protein, 465 aa, Artificial Sequence
  Synthetic polypeptide
MEPSSLELPADTVQRIAAELKCHPTDERVALHLDEEDKLRHFRECFYIPKIQDLPPVDLSLVNKDENAIYFLGNSLGLQPKMVKTYLEEELDKWAKIAVYGHEVGKRPWITADESIVGLMKDIVGANEKEIALMNALTVNLHLLMLSFFKPTPKRYKILLEAKAFPSDHYAIESQLQLHGLNIEESMRMIKPREGEETLRIEDILEVIEKEGDSIAVILFSGVHFYTGQHFNIPAITKAGQAKGCYVGFDLAHAVGNVELYLHDWGVDFACWCSYKYLNAGAGGIAGAFIHEKHAHTIKPALVGWYGHELSTRFKMDNKLQLIPGVCGFRISNPPIVLICSLHASLEIFKQATMKALRKKSVLLTGYLEYLIKHNYGKDKAATKKPVVNIITPSHVEERGCQLTFTFNVPNKDVFQELEKRGVVCDKRNPNGIRVAPVPLYNSFHDVYKFTNLLTSILDSAETKN

SEQ ID NO: 68 - protein, 465 aa, Artificial Sequence
  Synthetic polypeptide
MEPSSLELPADTVQRIAAELKCHPTDERVALHLDEEDKLRHFRECFYIPKIQDLPPVDLSLVNKDENAIYFLGNSLGLQPKMVKTYLEEELDKWAKIAVYGHEVGKRPWITADESIVGLMKDIVGANEKEIALMNALTVNLHLLMLSFFKPTPKRYKILLEAKAFPSDHYAIESQLQLHGLNIEESMRMIKPREGEETLRIEDILEVIEKEGDSIAVILFSGVHFYTGQHFNIPAITKAGQAKGCYVGFDLAHAVGNVELYLHDWGVDFACWCSYKYLNAGAGGIAGAFIHEKHAHTIKPALVGWYGHELSTRFKMDNKLQLIPGVCGFRISNPPILLACSLHASLEIFKQATMKALRKKSVLLTGYLEYLIKHNYGKDKAATKKPVVNIITPSHVEERGCQLTLTFNVPNKDVFQELEKRGVVCDKRNPNGIRVAPVPLYNSFHDVYKFTNLLTSILDSAETKN

SEQ ID NO: 69 - protein, 465 aa, Artificial Sequence
  Synthetic polypeptide
MEPSSLELPADTVQRIAAELKCHPTDERVALHLDEEDKLRHFRECFYIPKIQDLPPVDLSLVNKDENAIYFLGNSLGLQPKMVKTYLEEELDKWAKIAVYGHEVGKRPWITADESIVGLMKDIVGANEKEIALMNALSVNLHLLMLSFFKPTPKRYKILLEAKAFPSDHYAIESQLQLHGLNIEESMRMIKPREGEETLRIEDILEVIEKEGDSIAVILFSGVHFYTGQHFNIPAITKAGQAKGCYVGFDLAHAVGNVELYLHDWGVDFACWCSYKYLNAGAGGIAGAFIHEKHAHTIKPALVGWFGHELSTRFKMDNKLQLIPGVCGFRISNPPILLACSLHASLEIFKQATMKALRKKSVLLTGYLEYLIKHNYGKDKAATKKPVVNIITPSHVEERGCQLTFTFSVPNKDVFQELEKRGVVCDKRNPNGIRVAPVPLYNSFHDVYKFTNLLTSILDSAETKN

SEQ ID NO: 70 - protein, 465 aa, Artificial Sequence
  Synthetic polypeptide
MEPSSLELPADTVQRIAAELKCHPTDERVALHLDEEDKLRHFRECFYIPKIQDLPPVDLSLVNKDENAIYFLGNSLGLQPKMVKTYLEEELDKWAKIAAYGHEVGKRPWITGDESIVGLMKDIVGANEKEIALMNALTVNLHLLMLSFFKPTPKRYKILLEAKAFPSDHYAIESQLQLHGLNIEESMRMIKPREGEETLRIEDILEVIEKEGDSIAVILFSGVHFYTGQHFNIPAITKAGQAKGCYVGFDLAHAVGNVELYLHDWGVDFACWCSYKYLNAGAGGIAGAFIHEKHAHTIKPALVGWIGHELSTRFKMDNKLQLIPGVCGFRISNPPIVLICSLHASLEIFKQATMKALRKKSVLLTGYLEYLIKHNYGKDKAATKKPVVNIITPSHVEERGCQLTFTFTVPNKDVFQELEKRGVVCDKRNPNGIRVAPVPLYNSFHDVYKFTNLLTSILDSAETKN

SEQ ID NO: 71 - protein, 465 aa, Artificial Sequence
  Synthetic polypeptide
MEPSSLELPADTVQRIAAELKCHPTDERVALHLDEEDKLRHFRECFYIPKIQDLPPVDLSLVNKDENAIYLLGNSLGLQPKMVKTYLEEELDKWAKIAIYGHEVGKRPWITGDESIVGLMKDIVGANEKEIALMNALTVNLHLLMLSFFKPTPKRYKILLEAKAFPSDHYAIESQLQLHGLNIEESMRMIKPREGEETLRIEDILEVIEKEGDSIAVILFSGVHFYTGQHFNIPAITKAGQAKGCYVGFDLAHAVGNVPLYLHDWGVDFACWCSYKYLNAGAGGIAGAFIHEKHAHTIKPALVGWFGHELSTRFKMDNKLQLIPGVCGFRISNPPILLVCSLHASLEIFKQATMKALRKKSVLLTGYLEYLIKHNYGKDKAATKKPVVNIITPSHVEERGCQLTITFSVPNKDVFQELEKRGVVCDKRNPNGIRVAPVPLYNSFHDVYKFTNLLTSILDSAETKN

SEQ ID NO: 72 - protein, 465 aa, Artificial Sequence
  Synthetic polypeptide
MEPSSLELPADTVQRIAAELKCHPTDERVALHLDEEDKLRHFRECFYIPKIQDLPPVDLSLVNKDENAIYLLGNSLGLQPKMVKTYLEEELDKWAKIAIYGHEVGKRPWITGDESIVGLMKDIVGANEKEVALMNALTVNLHLLMLSFFKPTPKRYKILLEAKAFPSDHYAIESQLQLHGLNIEESMRMIKPREGEETLRIEDILEVIEKEGDSIAVILFSGVHFYTGQHFNIPAITKAGQAKGCYVGFDLAHAVGNVPLYLHDWGVDFACWCSYKYLNAGPGGIAGAFIHEKHAHTIKPALVGWFGHELSTRFKMDNKLQLIPGVCGFRISNPPILLVCSLHASLEIFKQATMKALRKKSVLLTGYLEYLIKHNYGKDKAATKKPVVNIITPSHVEERGCQLTITFSVPNKDVFQELEKRGVVCDKRNPNGIRVAPVPLYNSFHDVYKFTNLLTSILDSAETKN

SEQ ID NO: 73 - protein, 465 aa, Artificial Sequence
  Synthetic polypeptide
MEPSSLELPADTVQRIAAELKCHPTDERVALHLDEEDKLRHFRECFYIPKIQDLPPVDLSLVNKDENAIYLLGNSLGLQPKMVKTYLEEELDKWAKIAIYGHEVGKRPWITGDESIVGLMKDIVGANEKEVALMNALTVNLHLLMLSFFKPTPKRYKILLEAKAFPSDHYAIESQLQLHGLNIEESMRMIKPREGEETLRIEDILEVIEKEGDSIAVILFSGVHFYTGQHFNIPAITKAGQAKGCYVGFDLAHAVGNVPLYLHDWGVDFACWCSYKYLNAGAGGIAGAFIHEKHAHTIKPALSGWFGHELSTRFKMDNKLQLIPGVCGFRISNPPILLVCSLHASLEIFKQATMKALRKKSVLLTGYLEYLIKHNYGKDKAATKKPVVNIITPSHVEERGCQLTITFSVPNKDVFQELEKRGVVCDKRNPNGIRVAPVPLYNSFHDVYKFTNLLTSILDSAETKN

SEQ ID NO: 74 - protein, 465 aa, Artificial Sequence
  Synthetic polypeptide
MEPSSLELPADTVQRIAAELKCHPTDERVALHLDEEDKLRHFRECFYIPKIQDLPPVDLSLVNKDENAIYLLGNSLGLQPKMVKTYLEEELDKWAKIAIYGHEVGKRPWITGDESIVGLMKDIVGANEKEVALMNALTVNLHLLMLSFFKPTPKRYKILLEAKAFPSDHYAIESQLQLHGLNIEESMRMIKPREGEETLRIEDILEVIEKEGDSIAVILFSGVHFYTGQHFNIPAITKAGQAKGCYVGWDLAHAVGNVELYLHDWGVDFACWCSYKYLNAGAGGIAGAFIHEKHAHTIKPALVGWFGHELSTRFKMDNKLQPIPGVCGFRISNPPILLVCSLHASLEIFKQATMKALRKKSVLLTGYLEYLIKHNYGKDKAATKKPVVNIITPSHVEERGCQLTITFSVPNKDVFQELEKRGVVCDKRNPNGIRVAPVPLYNSFHDVYKFTNLLTSILDSAETKN

SEQ ID NO: 75 - protein, 465 aa, Artificial Sequence
  Synthetic polypeptide
MEPSSLELPADTVQRIAAELKCHPTDERVALHLDEEDKLRHFRECFYIPKIQDLPPVDLSLVNKDENAIYLLGNSLGLQPKMVKTYLEEELDKWAKIAAYGHEVGKRPWITGDESIVGLMKDIVGANEKEIALMNALTVNLHLLMLSFFKPTPKRYKILLEAKAFPSDHYAIESQLQLHGLNIEESMRMIKPREGEETLRIEDILEVIEKEGDSIAVILFSGVHFYTGQHFNIPAITKAGQAKGCYVGFDLAHAVGNVPLYLHDWGVDFACWCSYKYLNAGAGGIAGAFIHEKHAHTIKPALVGWFGHELSTRFKMDNKLQPIPGVCGFRISNPPILLVCSLHASLEIFKQATMKALRKKSVLLTGYLEYLIKHNYGKDKAATKKPVVNIITPSHVEERGCQLTITFSVPNKDVFQELEKRGVVCDKRNPNGIRVAPVPLYNSFHDVYKFTNLLTSILDSAETKN

SEQ ID NO: 76 - protein, 465 aa, Artificial Sequence
  Synthetic polypeptide
MEPSSLELPADTVQRIAAELKCHPTDERVALHLDEEDKLRHFRECFYIPKIQDLPPVDLSLVNKDENAIYLLGNSLGLQPKMVKTYLEEELDKWAKIAAYGHEVGKRPWITGDESIVGLMKDIVGANEKEIALMNALTVNLHLLMLSFFKPTPKRYKILLEAKAFPSDHYAIESQLQLHGLNIEESMRMIKPREGEETLRIEDILEVIEKEGDSIAVILFSGVHFYTGQHFNIPAITKAGQAKGCYVGWDLAHAVGNVPLYLHDWGVDFACWCSYKYLNAGAGGIAGAFIHEKHAHTIKPALSGWFGHELSTRFKMDNKLQLIPGVCGFRISNPPILLVCSLHASLEIFKQATMKALRKKSVLLTGYLEYLIKHNYGKDKAATKKPVVNIITPSHVEERGCQLTITFSVPNKDVFQELEKRGVVCDKRNPNGIRVAPVPLYNSFHDVYKFTNLLTSILDSAETKN

SEQ ID NO: 77 - protein, 465 aa, Artificial Sequence
  Synthetic polypeptide
MEPSSLELPADTVQRIAAELKCHPTDERVALHLDEEDKLRHFRECFYIPKIQDLPPVDLSLVNKDENAIYFLGNSLGLQPKMVKTYLEEELDKWAKIAAYGHEVGKRPWITADESIVGLMKDIVGANEKEIALMNALTVNLHLLMLSFFKPTPKRYKILLEAKAFPSDHYAIESQLQLHGLNIEESMRMIKPREGEETLRIEDILEVIEKEGDSIAVILFSGVHFYTGQHFNIPAITKAGQAKGCYVGFDLAHAVGNVELYLHDWGVDFACWCSYKYLNAGAGGIAGAFIHEKHAHTIKPALVGWYGHELSTRFKMDNKLQLIPGVCGFRISNPPIVLVCSLHASLEIFKQATMKALRKKSVLLTGYLEYLIKHNYGKDKAATKKPVVNIITPSHVEERGCQLTLTFSVPNKDVFQELEKRGVVCDKRNPNGIRVAPVPLYNSFHDVYKFTNLLTSILDSAETKN

SEQ ID NO: 78 - protein, 465 aa, Artificial Sequence
  Synthetic polypeptide
MEPSSLELPADTVQRIAAELKCHPTDERVALHLDEEDKLRHFRECFYIPKIQDLPPVDLSLVNKDENAIYFLGNSLGLQPKMVKTYLEEELDKWAKIAAYGHEVGKRPWITADESIVGLMKDIVGANEKEIALMNALTVNLHLLMLSFFKPTPKRYKILLEAKAFPSDHYAIESQLQLHGLNIEESMRMIKPREGEETLRIEDILEVIEKEGDSIAVILFSGVHFYTGQHFNIPAITKAGQAKGCYVGFDLAHAVGNVELYLHDWGVDFACWCSYKYLNAGAGGIAGAFIHEKHAHTIKPALVGWYGHELSTRFKMDNKLQLIPGVCGFRISNPPILLMCSLHASLEIFKQATMKALRKKSVLLTGYLEYLIKHNYGKDKAATKKPVVNIITPSHVEERGCQLTLTFSVPNKDVFQELEKRGVVCDKRNPNGIRVAPVPLYNSFHDVYKFTNLLTSILDSAETKN

SEQ ID NO: 79 - protein, 465 aa, Artificial Sequence
  Synthetic polypeptide
MEPSSLELPADTVQRIAAELKCHPTDERVALHLDEEDKLRHFRECFYIPKIQDLPPVDLSLVNKDENAIYFLGNSLGLQPKMVKTYLEEELDKWAKIAAYGHEVGKRPWITADESIVGLMKDIVGANEKEIALMNALTVNLHLLMLSFFKPTPKRYKILLEAKAFPSDHYAIESQLQLHGLNIEESMRMIKPREGEETLRIEDILEVIEKEGDSIAVILFSGVHFYTGQHFNIPAITKAGQAKGCYVGFDLAHAVGNVELYLHDWGVDFACWCSYKYLNAGAGGIAGAFIHEKHAHTIKPALVGWYGHELSTRFKMDNKLQLIPGVCGFRISNPPILLSCSLHASLEIFKQATMKALRKKSVLLTGYLEYLIKHNYGKDKAATKKPVVNIITPSHVEERGCQLTLTFSVPNKDVFQELEKRGVVCDKRNPNGIRVAPVPLYNSFHDVYKFTNLLTSILDSAETKN

SEQ ID NO: 80 - protein, 465 aa, Artificial Sequence
  Synthetic polypeptide
MEPSSLELPADTVQRIAAELKCHPTDERVALHLDEEDKLRHFRECFYIPKIQDLPPVDLSLVNKDENAIYFLGNSLGLQPKMVKTYLEEELDKWAKIAAYGHEVGKRPWITSDESIVGLMKDIVGANEKEIALMNALTVNLHLLMLSFFKPTPKRYKILLEAKAFPSDHYAIESQLQLHGLNIEESMRMIKPREGEETLRIEDILEVIEKEGDSIAVILFSGVHFYTGQHFNIPAITKAGQAKGCYVGFDLAHAVGNVELYLHDWGVDFACWCSYKYLNAGAGGIAGAFIHEKHAHTIKPALVGWLGHELSTRFKMDNKLQLIPGVCGFRISNPPILLTCSLHASLEIFKQATMKALRKKSVLLTGYLEYLIKHNYGKDKAATKKPVVNIITPSHVEERGCQLTITFTVPNKDVFQELEKRGVVCDKRNPNGIRVAPVPLYNSFHDVYKFTNLLTSILDSAETKN

SEQ ID NO: 81 - protein, 465 aa, Artificial Sequence
  Synthetic polypeptide
MEPSSLELPADTVQRIAAELKCHPTDERVALHLDEEDKLRHFRECFYIPKIQDLPPVDLSLVNKDENAIYFLGNSLGLQPKMVKTYLEEELDKWAKIAAYGHEVGKRPWITSDESIVGLMKDIVGANEKEIALMNALTVNLHLLMLSFFKPTPKRYKILLEAKAFPSDHYAIESQLQLHGLNIEESMRMIKPREGEETLRIEDILEVIEKEGDSIAVILFSGVHFYTGQHFNIPAITKAGQAKGCYVGFDLAHAVGNVELYLHDWGVDFACWCSYKYLNAGAGGIAGAFIHEKHAHTIKPALVGWYGHELSTRFKMDNKLQLIPGVCGFRISNPPILLTCSLHASLEIFKQATMKALRKKSVLLTGYLEYLIKHNYGKDKAATKKPVVNIITPSHVEERGCQLTLTFSVPNKDVFQELEKRGVVCDKRNPNGIRVAPVPLYNSFHDVYKFTNLLTSILDSAETKN

SEQ ID NO: 82 - protein, 465 aa, Artificial Sequence
  Synthetic polypeptide
MEPSSLELPADTVQRIAAELKCHPTDERVALHLDEEDKLRHFRECFYIPKIQDLPPVDLSLVNKDENAIYFLGNSLGLQPKMVKTYLEEELDKWAKIAAYGHEVGKRPWLTGDESIVGLMKDIVGANEKEIALMNALTVNLHLLMLSFFKPTPKRYKILLEAKAFPSDHYAIESQLQLHGLNIEESMRMIKPREGEETLRIEDILEVIEKEGDSIAVILFSGVHFYTGQHFNIPAITKAGQAKGCYVGFDLAHAVGNVELYLHDWGVDFACWCSYKYLNAGAGGIAGAFIHEKHAHTIKPALVGWFGHELSTRFKMDNKLQLIPGVCGFRISNPPILLVCSLHASLEIFKQATMKALRKKSVLLTGYLEYLIKHNYGKDKAATKKPVVNIITPSHVEERGCQLTITFSVPNKDVFQELEKRGVVCDKRNPNGIRVAPVPLYNSFHDVYKFTNLLTSILDSAETKN

SEQ ID NO: 83 - protein, 465 aa, Artificial Sequence
  Synthetic polypeptide
MEPSSLELPADTVQRIAAELKCHPTDERVALHLDEEDKLRHFRECFYIPKIQDLPPVDLSLVNKDENAIYFLGNSLGLQPKMVKTYLEEELDKWAKIAAYGHEVGKRPWLTGDESIVGLMKDIVGANEKEIALMNALTVNLHLLMLSFFKPTPKRYKILLEAKAFPSDHYAIESQLQLHGLNIEESMRMIKPREGEETLRIEDILEVIEKEGDSIAVILFSGVHFYTGQHFNIPAITKAGQAKGCYVGFDLAHAVGNVELYLHDWGVDFACWCSYKYLNAGAGGIAGAFIHEKHAHTIKPALVGWLGHELSTRFKMDNKLQLIPGVCGFRISNPPILLVCSLHASLEIFKQATMKALRKKSVLLTGYLEYLIKHNYGKDKAATKKPVVNIITPSHVEERGCQLTITFSVPNKDVFQELEKRGVVCDKRNPNGIRVAPVPLYNSFHDVYKFTNLLTSILDSAETKN

SEQ ID NO: 84 - protein, 465 aa, Artificial Sequence
  Synthetic polypeptide
MEPSSLELPADTVQRIAAELKCHPTDERVALHLDEEDKLRHFRECFYIPKIQDLPPVDLSLVNKDENAIYFLGNSLGLQPKMVKTYLEEELDKWAKIAAYGHEVGKRPWITGDESIVGLMKDIVGANEKEMALMNALTVNLHLLMLSFFKPTPKRYKILLEAKAFPSDHYAIESQLQLHGLNIEESMRMIKPREGEETLRIEDILEVIEKEGDSIAVILFSGVHFYTGQHFNIPAITKAGQAKGCYVGWDLAHAVGNVELYLHDWGVDFACWCGYKYLNAGAGGIAGAFIHEKHAHTIKPALVGWFGHELSTRFKMDNKLQLIPGVCGFRISNPPILLVCSLHASLEIFKQATMKALRKKSVLLTGYLEYLIKHNYGKDKAATKKPVVNIITPSHVEERGCQLTITFSVPNKDVFQELEKRGVVCDKRNPNGIRVAPVPLYNSFHDVYKFTNLLTSILDSAETKN

SEQ ID NO: 85 - protein, 465 aa, Artificial Sequence
  Synthetic polypeptide
MEPSSLELPADTVQRIAAELKCHPTDERVALHLDEEDKLRHFRECFYIPKIQDLPPVDLSLVNKDENAIYFLGNSLGLQPKMVKTYLEEELDKWAKIAAYGHEVGKRPWITGDESIVGLMKDIVGANEKEVALMNALTVNLHLLMLSFFKPTPKRYKILLEAKAFPSDHYAIESQLQLHGLNIEESMRMIKPREGEETLRIEDILEVIEKEGDSIAVILFSGVHFYTGQHFNIPAITKAGQAKGCYVGWDLAHAVGNVELYLHDWGVDFACWCSYKYLNAGAGGIAGAFIHEKHAHTIKPALVGWFGHELSTRFKMDNKLQLIPGVCGFRISNPPILLVCSLHASLEIFKQATMKALRKKSVLLTGYLEYLIKHNYGKDKAATKKPVVNIITPSHVEERGCQLTITFSVPNKDVFQELEKRGVVCDKRNPNGIRVAPVPLYNSFHDVYKFTNLLTSILDSAETKN

SEQ ID NO: 86 - protein, 465 aa, Artificial Sequence
  Synthetic polypeptide
MEPSSLELPADTVQRIAAELKCHPTDERVALHLDEEDKLRHFRECFYIPKIQDLPPVDLSLVNKDENAIYFLGNSLGLQPKMVKTYLEEELDKWAKIAAYGHEVGKRPWITGDESIVGLMKDIVGANEKEIALMNALSVNLHLLMLSFFKPTPKRYKILLEAKAFPSDHYAIESQLQLHGLNIEESMRMIKPREGEETLRIEDILEVIEKEGDSIAVILFSGVHFYTGQHFNIPAITKAGQAKGCYVGFDLAHAVGNVELYLHDWGVDFACWCSYKYLNAGAGGIAGAFIHEKHAHTIKPALVGWFGHELSTRFKMDNKLQLIPGVCGFRISNPPILLVCSLHASLEIFKQATMKALRKKSVLLTGYLEYLIKHNYGKDKAATKKPVVNIITPSHVEERGCQLTITFSVPNKDVFQELEKRGVVCDKRNPNGIRVAPVPLYNSFHDVYKFTNLLTSILDSAETKN

SEQ ID NO: 87 - protein, 465 aa, Artificial Sequence
  Synthetic polypeptide
MEPSSLELPADTVQRIAAELKCHPTDERVALHLDEEDKLRHFRECFYIPKIQDLPPVDMSLVNKDENAIYFLGNSLGLQPKMVKTYLEEELDKWAKIAAYGHEVGKRPWITSDESIVGLMKDIVGANEKEIALMNALTVNLHLLMLSFFKPTPKRYKILLEAKAFPSDHYAIESQLQLHGLNIEESMRMIKPREGEETLRIEDILEVIEKEGDSIAVILFSGVHFYTGQHFNIPAITKAGQAKGCYVGFDLAHAVGNVELYLHDWGVDFACWCSYKYLNAGAGGIAGAFIHEKHAHTIKPALVGWYGHELSTRFKMDNKLQLIPGVCGFRISNPPILLACSLHASLEIFKQATMKALRKKSVLLTGYLEYLIKHNYGKDKAATKKPVVNIITPSHVEERGCQLTLTFNVPNKDVFQELEKRGVVCDKRNPNGIRVAPVPLYNSFHDVYKFTNLLTSILDSAETKN

SEQ ID NO: 88 - protein, 465 aa, Artificial Sequence
  Synthetic polypeptide
MEPSSLELPADTVQRIAAELKCHPTDERVALHLDEEDKLRRFRECFYIPKIQDLPPVDLSLVNKDENAIYFLGNSLGLQPKMVKTYLEEELDKWAKIAAYGHEVGKRPWITGDESIVGLMKDIVGANEKEIALMNALTVNLHLLMLSFFKPTPKRYKILLEAKAFPSDHYAIESLLQLHGLNIEESMRMIKPREGEETLRIEDILEVIEKEGDSIAVILFSGVHFYTGQHFNIPAITKAGQAKGCYVGFDLAHAVGNVELYLHDWGVDFACWCSYKYLNAGAGGIAGAFIHEKHAHTIKPALVGWFGHELSTRFKMDNKLQLIPGVCGFRISNPPILLVCSLHASLEIFKQATMKALRKKSVLLTGYLEYLIKHNYGKDKAATKKPVVNIITPSHVEERGCQLTITFSVPNKDVFQELEKRGVVCDKRNPNGIRVTPVPLYNSFHDVYKFTNLLTSILDSAETKN

SEQ ID NO: 89 - protein, 465 aa, Artificial Sequence
  Synthetic polypeptide
MEPSSLELPADTVQRIAAELKCHPTDERVALHLDEEDKLRHFRECFYIPKIQDLPPVDLSLVNKDENAIYFLGNSLGLQPKMVKTYLEEELDKWAKIAAYGHEVGKRPWITGDESIVGLMKDIVGANEKEIALMNALSVNLHLLMLSFFKPTPKRYKILLEAKAFPSDHYAIESQLQLHGLNIEESMRMIKPREGEETLRIEDILEVIEKEGDSIAVILFSGVHFYTGQHFNIPAITKAGQAKGCYVGFDLAHAVGNVELYLHDWGVDFACWCSYKYLNAGAGGIAGAFIHEKHAHTIKPALVGWFGHELSTRFKMDNKLQLIPGVCGFRISNPPILLVCSLHASLEIFKQATMKALRKKSVLLTGYLEYLIKHNYGKDKAATKKPVVNIITPSHVEERGCQLTITFSVPNKDVFQELEKRGVVCDKRNPNGIRVTPVPLYNSFHDVYKFTNLLTSILDSAETKN

SEQ ID NO: 90 - protein, 465 aa, Artificial Sequence
  Synthetic polypeptide
MEPSSLELPADTVQRIAAELKCHPTDERVALHLDEEDKLRHFRECFYIPKIQDLPPVDLSLVNKDENAIYLLGNSLGLQPKMVKTYLEEELDKWAKIAIYGHEVGKRPWITADESIVGLMKDIVGANEKEIALMNALSVNLHLLMLSFFKPTPKRYKILLEAKAFPSDHYAIESQLQLHGLNIEESMRMIKPREGEETLRIEDILEVIEKEGDSIAVILFSGVHFYTGQHFNIPAITKAGQAKGCYVGFDLAHAVGNVELYLHDWGVDFACWCSYKYLNAGAGGIAGAFIHEKHAHTIKPALVGWYGHELSTRFKMDNKLQLIPGVCGFRISNPPIVLICSLHASLEIFKQATMKALRKKSVLLTGYLEYLIKHNYGKDKAATKKPVVNIITPSHVEERGCQLTLTFNVPNKDVFQELEKRGVVCDKRNPNGIRVTPVPLYNSFHDVYKFTNLLTSILDSAETKN

SEQ ID NO: 91 - protein, 465 aa, Artificial Sequence
  Synthetic polypeptide
MEPSSLELPADTVQRIAAELKCHPTDERVALHLDEEDKLRHFRECFYIPKIQDLPPVDLSLVNKDENAIYFLGNSLGLQPKMVKTYLEEELDKWAKIAAYGHEVGKRPWITGDESIVGLMKDIVGANEKEIALMNALTVNLHLLMLSFFKPTPKRYKILLEAKAFPSDHYAIESQLQLHGLNIEESMRMIKPREGEETLRIEDILEVIEKEGDSIAVILFSGVHFYTGQHFNIPAITKAGQAKGCYVGFDLAHAVGNVELYLHDWGVDFACWCSYKYLNAGAGGIAGAFIHEKHAHTIKPALVGWYGHELSTRFKMDNKLQLIPGVCGFRISNPPILLVCSLHASLEIFKQATMKALRKKSVLLTGYLEYLIKHNYGKDKAATKKPVVNIITPSHVEERGCQLTITFSVPNKDVFQELEKRGVVCDKRNPNGIRVAPVPLYNSFHDVYKFTNLLTSILDSAETKN

SEQ ID NO: 92 - protein, 465 aa, Artificial Sequence
  Synthetic polypeptide
MEPSSLELPADTVQRIAAELKCHPTDERVALHLDEEDKLRHFRECFYIPKIQDLPPVDLSLVNKDENAIYLLGNSLGLQPKMVKTYLEEELDKWAKIAIYGHEVGKRPWITGDESIVGLMKDIVGANEKEIALMNALTVNLHLLMLSFFKPTPKRYKILLEAKAFPTDHYAIESQLQLHGLNIEESMRMIKPREGEETLRIEDILEVIEKEGDSIAVILFSGVHFYTGQHFNIPAITKAGQAKGCYVGFDLAHAVGNVPLYLHDWGVDFACWCSYKYLNAGAGGIAGAFIHEKHAHTIKPALVGWFGHELSTRFKMDNKLQLIPGVCGFRISNPPILLVCSLHASLEIFKQATMKALRKKSVLLTGYLEYLIKHNYGKDKAATKKPVVNIITPSHVEERGCQLTITFSVPNKDVFQELEKRGVVCDKRNPNGIRVAPVPLYNSFHDVYKFTNLLTSILDSAETKN

SEQ ID NO: 93 - protein, 465 aa, Artificial Sequence
  Synthetic polypeptide
MEPSSLELPADTVQRIAAELKCHPTDERVALHLDEEDKLRHFRECFYIPKIQDLPPVDLSLVNKDENAIYFLGNSLGLQPKMVKTYLEEELDKWAKIAIYGHEVGKRPWITADESIVGLMKDIVGANEKEIALMNALTVNLHLLMLSFFKPTPKRYKILLEAKAFPSDHYAIESQLQLHGLNIEESMRMIKPREGEETLRIEDILEVIEKEGDSIAVILFSGVHFYTGQHFNIPAITKAGQAKGCYVGFDLAHAVGNVELYLHDWGVDFACWCSYKYLNAGAGGIAGAFIHEKHAHTIKPALVGWYGHELSTRFKMDNKLQLIPGVCGFRISNPPILLVCSLHASLEIFKQATMKALRKKSVLLTGYLEYLIKHNYGKDKAATKKPVVNIITPSHVEERGCQLTLTFNVPNKDVFQELEKRGVVCDKRNPNGIRVTPVPLYNSFHDVYKFTNLLTSILDSAETKN